European Patent Specification EP 4 199 946 B1, published June 5, 2024. Title: CRF2 RECEPTOR AGONISTS AND THEIR USE IN THERAPY. Applicant: SANOFI. The sequence listing filed with the application follows.

SEQUENCE LISTING (227 sequences)

SEQ ID NO: 1 - protein, 38 aa, Artificial Sequence
  compound Seq_1
  VARIANT 12: K* denotes the modified lysine residue at X12, Ra denotes the albumin-binding moiety, Ra is "-gGlu-C(O)(CH2)14CH3
  MOD_RES 38: C-terminal amino acid residue is amidated as a primary amide
IVLSLDVPIGLKQILLEQEKQEKEKQQAETNAQILAQV

SEQ ID NO: 2 - protein, 38 aa, Artificial Sequence
  compound Seq_2
  VARIANT 12: K* denotes the modified lysine residue at X12, Ra denotes the albumin-binding moiety, Ra is "-gGlu-C(O)(CH2)14CH3
  MOD_RES 38: C-terminal amino acid residue is amidated as a primary amide
IVLSLDVPIKLKKILLEQEKQEKEKQQAETNAQILAQV

SEQ ID NO: 3 - protein, 38 aa, Artificial Sequence
  compound Seq_3
  VARIANT 12: K* denotes the modified lysine residue at X12, Ra denotes the albumin-binding moiety, Ra is "-gGlu-C(O)(CH2)14CH3
  MOD_RES 38: C-terminal amino acid residue is amidated as a primary amide
IVLSLDVPIKLKKILLEQEKQEKEKQQAEKNAQILAQV

SEQ ID NO: 4 - protein, 38 aa, Artificial Sequence
  compound Seq_4
  VARIANT 12: K* denotes the modified lysine residue at X12, Ra denotes the albumin-binding moiety, Ra is "-gGlu-C(O)(CH2)14CH3
  MOD_RES 38: C-terminal amino acid residue is amidated as a primary amide
IVLSLDVPIGLKQKLLKQEKQEKEKQQAETNAKILAQV

SEQ ID NO: 5 - protein, 38 aa, Artificial Sequence
  compound Seq_5
  VARIANT 12: K* denotes the modified lysine residue at X12, Ra denotes the albumin-binding moiety, Ra is "-gGlu-C(O)(CH2)14CH3
  MOD_RES 38: C-terminal amino acid residue is amidated as a primary amide
IVLSLDVPIGLKQKLLKQQRQRKERQQAETNARILARV

SEQ ID NO: 6 - protein, 38 aa, Artificial Sequence
  compound Seq_6
  VARIANT 12: K* denotes the modified lysine residue at X12, Ra denotes the albumin-binding moiety, Ra is "-gGlu-C(O)(CH2)14CH3
  MOD_RES 38: C-terminal amino acid residue is amidated as a primary amide
IVLSLDVPIGLKQKLLKQQRQRKERQQAEKNARILARV

SEQ ID NO: 7 - protein, 38 aa, Artificial Sequence
  compound Seq_7
  VARIANT 7: D-valine (v)
  VARIANT 12: K* denotes the modified lysine residue at X12, Ra denotes the albumin-binding moiety, Ra is "-gGlu-C(O)(CH2)14CH3
  MOD_RES 38: C-terminal amino acid residue is amidated as a primary amide
IVLSLDXPTKLKQKLLKQERQRKEREQAEKNARILARV

SEQ ID NO: 8 - protein, 38 aa, Artificial Sequence
  compound Seq_8
  VARIANT 12: K* denotes the modified lysine residue at X12, Ra denotes the albumin-binding moiety, Ra is "-gGlu-C(O)(CH2)14CH3
  MOD_RES 38: C-terminal amino acid residue is amidated as a primary amide
FTLSLDVPTKIKQKLLKQEKQKKQRQKAKTAAQILAQV

SEQ ID NO: 9 - protein, 38 aa, Artificial Sequence
  compound Seq_9
  VARIANT 12: K* denotes the modified lysine residue at X12, Ra denotes the albumin-binding moiety, Ra is "-gGlu-C(O)(CH2)14CH3
  MOD_RES 38: C-terminal amino acid residue is amidated as a primary amide
FTLSLDVPTKIKQKLLKQEKQKKQRQKAKTAKQILEQV

SEQ ID NO: 10 - protein, 38 aa, Artificial Sequence
  compound Seq_10
  VARIANT 12: K* denotes the modified lysine residue at X12, Ra denotes the albumin-binding moiety, Ra is "-gGlu-C(O)(CH2)14CH3
  MOD_RES 38: C-terminal amino acid residue is amidated as a primary amide
FTLSLDVPTKIKQKLLKQEKQKKQRQKAKTNKQILEQV

SEQ ID NO: 11 - protein, 38 aa, Artificial Sequence
  compound Seq_11
  VARIANT 12: K* denotes the modified lysine residue at X12, Ra denotes the albumin-binding moiety, Ra is "-gGlu-C(O)(CH2)14CH3
  MOD_RES 38: C-terminal amino acid residue is amidated as a primary amide
FTLSLDVPTKIKQKLLKQEKQKKQRQKAKTNAQILAQV

SEQ ID NO: 12 - protein, 38 aa, Artificial Sequence
  compound Seq_12
  VARIANT 12: K* denotes the modified lysine residue at X12, Ra denotes the albumin-binding moiety, Ra is "-gGlu-C(O)(CH2)14CH3
  MOD_RES 38: C-terminal amino acid residue is amidated as a primary amide
FTLSLDVPTKIKQKLLKQEKQRKQKQQAKTNAKILARV

SEQ ID NO: 13 - protein, 38 aa, Artificial Sequence
  compound Seq_13
  VARIANT 12: K* denotes the modified lysine residue at X12, Ra denotes the albumin-binding moiety, Ra is "-{AEEA}2-gGlu-C(O)(CH2)16COOH
  MOD_RES 38: C-terminal amino acid residue is amidated as a primary amide
FTLSLDVPTKIKQILFKQQKQKKERQQAEKNKQLLEQI

SEQ ID NO: 14 - protein, 38 aa, Artificial Sequence
  compound Seq_14
  VARIANT 12: K* denotes the modified lysine residue at X12, Ra denotes the albumin-binding moiety, Ra is "-gGlu-C(O)(CH2)14CH3
  MOD_RES 38: C-terminal amino acid residue is amidated as a primary amide
FTLSLDVPTKIKQKLLKQEKQRKQKQKAKTNAKILARV

SEQ ID NO: 15 - protein, 38 aa, Artificial Sequence
  compound Seq_15
  VARIANT 12: K* denotes the modified lysine residue at X12, Ra denotes the albumin-binding moiety, Ra is "-gGlu-C(O)(CH2)14CH3
  MOD_RES 38: C-terminal amino acid residue is amidated as a primary amide
FTLSLDVPTKIKQKLFKQAKQKKQRQKAKTNAQILARV

SEQ ID NO: 16 - protein, 38 aa, Artificial Sequence; identical to SEQ ID NO: 6
  compound Seq_16
  VARIANT 12: K* denotes the modified lysine residue at X12, Ra denotes the albumin-binding moiety, Ra is "-{AEEA}2-gGlu-C(O)(CH2)16COOH
  MOD_RES 38: C-terminal amino acid residue is amidated as a primary amide

SEQ ID NO: 17 - protein, 38 aa, Artificial Sequence
  compound Seq_17
  VARIANT 12: K* denotes the modified lysine residue at X12, Ra denotes the albumin-binding moiety, Ra is "-gGlu-C(O)(CH2)14CH3
  MOD_RES 38: C-terminal amino acid residue is amidated as a primary amide
IVLSLDVPIKLKKILLEQEKQKKQREQAETNKQILAQV

SEQ ID NO: 18 - protein, 38 aa, Artificial Sequence
  compound Seq_18
  VARIANT 7: D-valine (v)
  VARIANT 12: K* denotes the modified lysine residue at X12, Ra denotes the albumin-binding moiety, Ra is "-gGlu-C(O)(CH2)14CH3
  MOD_RES 38: C-terminal amino acid residue is amidated as a primary amide
IVLSLDXPTKLKQKLLKQERQRKEREQAEKNKRILERV

SEQ ID NO: 19 - protein, 38 aa, Artificial Sequence
  compound Seq_19
  VARIANT 7: D-valine (v)
  VARIANT 12: K* denotes the modified lysine residue at X12, Ra denotes the albumin-binding moiety, Ra is "-gGlu-C(O)(CH2)14CH3
  VARIANT 23: 2-aminoisobutyric acid (Aib)
  MOD_RES 38: C-terminal amino acid residue is amidated as a primary amide
IVLSLDXPTKLKQKLLKQERQRXEREQAEKNKRILERV

SEQ ID NO: 20 - protein, 38 aa, Artificial Sequence
  compound Seq_20
  VARIANT 7: D-valine (v)
  VARIANT 12: K* denotes the modified lysine residue at X12, Ra denotes the albumin-binding moiety, Ra is "-gGlu-C(O)(CH2)14CH3
  VARIANT 24: 2-aminoisobutyric acid (Aib)
  MOD_RES 38: C-terminal amino acid residue is amidated as a primary amide
IVLSLDXPTKLKQKLLKQERQRKXREQAEKNKRILERV

SEQ ID NO: 21 - protein, 38 aa, Artificial Sequence
  compound Seq_21
  VARIANT 7: D-valine (v)
  VARIANT 12: K* denotes the modified lysine residue at X12, Ra denotes the albumin-binding moiety, Ra is "-gGlu-C(O)(CH2)14CH3
  VARIANT 24: 2-aminoisobutyric acid (Aib)
  MOD_RES 38: C-terminal amino acid residue is amidated as a primary amide
IVLSLDXPTKLKQKLLKQERQRKEXEQAEKNKRILERV

SEQ ID NO: 22 - protein, 38 aa, Artificial Sequence
  compound Seq_22
  VARIANT 12: K* denotes the modified lysine residue at X12, Ra denotes the albumin-binding moiety, Ra is "-{AEEA}2-gGlu-C(O)(CH2)16COOH
  VARIANT 23: 2-aminoisobutyric acid (Aib)
  MOD_RES 38: C-terminal amino acid residue is amidated as a primary amide
IVLSLDVPIKLKQILLKQERQKXQRQKAEKNKQILAQV

SEQ ID NO: 23 - protein, 38 aa, Artificial Sequence
  compound Seq_23
  VARIANT 7: D-valine (D)
  VARIANT 12: K* denotes the modified lysine residue at X12, Ra denotes the albumin-binding moiety, Ra is "-gGlu-C(O)(CH2)14CH3
  VARIANT 26: 2-aminoisobutyric acid (Aib)
  MOD_RES 38: C-terminal amino acid residue is amidated as a primary amide
IVLSLDXPTKLKQKLLKQERQRKERXQAEKNKRILERV

SEQ ID NO: 24 - protein, 38 aa, Artificial Sequence; identical to SEQ ID NO: 18
  compound Seq_24
  VARIANT 7: D-valine (v)
  VARIANT 12: K* denotes the modified lysine residue at X12, Ra denotes the albumin-binding moiety, Ra is "-{AEEA}2-gGlu-C(O)(CH2)16COOH
  MOD_RES 38: C-terminal amino acid residue is amidated as a primary amide

SEQ ID NO: 25 - protein, 38 aa, Artificial Sequence
  compound Seq_25
  VARIANT 7: D-valine (v)
  VARIANT 12: K* denotes the modified lysine residue at X12, Ra denotes the albumin-binding moiety, Ra is "-gGlu-C(O)(CH2)14CH3
  MOD_RES 38: C-terminal amino acid residue is amidated as a primary amide
IVLSLDXPTKLKKKLLKQERKRKEREKAEKNARILERV

SEQ ID NO: 26 - protein, 38 aa, Artificial Sequence
  compound Seq_26
  VARIANT 7: D-valine (v)
  VARIANT 12: K* denotes the modified lysine residue at X12, Ra denotes the albumin-binding moiety, Ra is "-gGlu-C(O)(CH2)14CH3
  VARIANT 27: 2-aminoisobutyric acid (Aib)
  MOD_RES 38: C-terminal amino acid residue is amidated as a primary amide
IVLSLDXPTKLKKKLLKQERKRKEREXAEKNARILERV

SEQ ID NO: 27 - protein, 38 aa, Artificial Sequence
  compound Seq_27
  VARIANT 7: D-valine (v)
  VARIANT 12: K* denotes the modified lysine residue at X12, Ra denotes the albumin-binding moiety, Ra is "-gGlu-C(O)(CH2)14CH3
  MOD_RES 38: C-terminal amino acid residue is amidated as a primary amide
IVLSLDXPTKLKKKLLKQERKRKEREQAEKNARILERV

SEQ ID NO: 28 - protein, 38 aa, Artificial Sequence
  compound Seq_28
  VARIANT 7: D-valine (d)
  VARIANT 12: K* denotes the modified lysine residue at X12, Ra denotes the albumin-binding moiety, Ra is "-gGlu-C(O)(CH2)14CH3
  MOD_RES 38: C-terminal amino acid residue is amidated as a primary amide
IVLSLDXPTKLKKKLLKQERKRKEREKAEKAARILERV

SEQ ID NO: 29 - protein, 38 aa, Artificial Sequence
  compound Seq_29
  VARIANT 7: D-valine (v)
  VARIANT 12: K* denotes the modified lysine residue at X12, Ra denotes the albumin-binding moiety, Ra is "-gGlu-C(O)(CH2)14CH3
  VARIANT 27: 2-aminoisobutyric acid (Aib)
  MOD_RES 38: C-terminal amino acid residue is amidated as a primary amide
IVLSLDXPTKLKKKLLKQERKRKEREXAEKAARILERV

SEQ ID NO: 30 - protein, 38 aa, Artificial Sequence
  compound Seq_30
  VARIANT 7: D-valine (v)
  VARIANT 12: K* denotes the modified lysine residue at X12, Ra denotes the albumin-binding moiety, Ra is "-gGlu-C(O)(CH2)14CH3
  MOD_RES 38: C-terminal amino acid residue is amidated as a primary amide
IVLSLDXPTKLKKKLLKQERKRKEREQAEKAARILERV

SEQ ID NO: 31 - protein, 38 aa, Artificial Sequence
  compound Seq_31
  VARIANT 7: D-valine (v)
  VARIANT 12: K* denotes the modified lysine residue at X12, Ra denotes the albumin-binding moiety, Ra is "-gGlu-C(O)(CH2)14CH3
  VARIANT 32: 2-aminoisobutyric acid (Aib)
  MOD_RES 38: C-terminal amino acid residue is amidated as a primary amide
IVLSLDXPTKLKQKLLKQERQRKEREQAEKNXRILERV

SEQ ID NO: 32 - protein, 38 aa, Artificial Sequence
  compound Seq_32
  VARIANT 7: D-valine (v)
  VARIANT 12: K* denotes the modified lysine residue at X12, Ra denotes the albumin-binding moiety, Ra is "-gGlu-C(O)(CH2)14CH3
  MOD_RES 38: C-terminal amino acid residue is amidated as a primary amide
IVLSLDXPTKLKQKLLKQERQRKEREQAEKNVRILERV

SEQ ID NO: 33 - protein, 38 aa, Artificial Sequence
  compound Seq_33
  VARIANT 7: D-valine (v)
  VARIANT 12: K* denotes the modified lysine residue at X12, Ra denotes the albumin-binding moiety, Ra is "-gGlu-C(O)(CH2)14CH3
  MOD_RES 38: C-terminal amino acid residue is amidated as a primary amide
IVLSLDXPTKLKQKLLKQERQRKEREQAEKNTRILERV

SEQ ID NO: 34 - protein, 38 aa, Artificial Sequence; identical to SEQ ID NO: 10
  compound Seq_34
  VARIANT 12: K* denotes the modified lysine residue at X12, Ra denotes the albumin-binding moiety, Ra is "-{AEEA}2-gGlu-C(O)(CH2)16COOH
  MOD_RES 38: C-terminal amino acid residue is amidated as a primary amide

SEQ ID NO: 35 - protein, 38 aa, Artificial Sequence; identical to SEQ ID NO: 17
  compound Seq_35
  VARIANT 12: K* denotes the modified lysine residue at X12, Ra denotes the albumin-binding moiety, Ra is "-{AEEA}2-gGlu-C(O)(CH2)16COOH
  MOD_RES 38: C-terminal amino acid residue is amidated as a primary amide

SEQ ID NO: 36 - protein, 38 aa, Artificial Sequence; identical to SEQ ID NO: 20
  compound Seq_36
  VARIANT 7: D-valine (v)
  VARIANT 12: K* denotes the modified lysine residue at X12, Ra denotes the albumin-binding moiety, Ra is "-{AEEA}2-gGlu-C(O)(CH2)16COOH
  VARIANT 24: 2-aminoisobutyric acid (Aib)
  MOD_RES 38: C-terminal amino acid residue is amidated as a primary amide

SEQ ID NO: 37 - protein, 38 aa, Artificial Sequence
  compound Seq_37
  VARIANT 12: K* denotes the modified lysine residue at X12, Ra denotes the albumin-binding moiety, Ra is "-{AEEA}2-gGlu-C(O)(CH2)16COOH
  MOD_RES 38: C-terminal amino acid residue is amidated as a primary amide
IVLSLDVPTKLKQKLLKQERQRKERQQAETNKRILERV

SEQ ID NO: 38 - protein, 38 aa, Artificial Sequence
  compound Seq_38
  VARIANT 12: K* denotes the modified lysine residue at X12, Ra denotes the albumin-binding moiety, Ra is "-{AEEA}2-gGlu-C(O)(CH2)16COOH
  VARIANT 23: 2-aminoisobutyric acid (Aib)
  MOD_RES 38: C-terminal amino acid residue is amidated as a primary amide
IVLSLDVPTKLKQKLLKQERQRXERQQAETNKRILERV

SEQ ID NO: 39 - protein, 38 aa, Artificial Sequence
  compound Seq_39
  VARIANT 12: K* denotes the modified lysine residue at X12, Ra denotes the albumin-binding moiety, Ra is "-{AEEA}2-gGlu-C(O)(CH2)16COOH
  MOD_RES 38: C-terminal amino acid residue is amidated as a primary amide
IVLSLDVPIKLKQILLEQERQRKERQQAETNAQILAQV

SEQ ID NO: 40 - protein, 38 aa, Artificial Sequence
  compound Seq_40
  VARIANT 12: K* denotes the modified lysine residue at X12, Ra denotes the albumin-binding moiety, Ra is "-{AEEA}2-gGlu-C(O)(CH2)16COOH
  MOD_RES 38: C-terminal amino acid residue is amidated as a primary amide
IVLSLDVPIKLKQILLEQERQRKERQQAETNVQILAQV

SEQ ID NO: 41 - protein, 38 aa, Artificial Sequence
  compound Seq_41
  VARIANT 12: K* denotes the modified lysine residue at X12, Ra denotes the albumin-binding moiety, Ra is "-{AEEA}2-gGlu-C(O)(CH2)16COOH
  MOD_RES 38: C-terminal amino acid residue is amidated as a primary amide
IVLSLDVPIKLKQILLEQERQRKERQQAEKNVRILERV

SEQ ID NO: 42 - protein, 38 aa, Artificial Sequence
  compound Seq_42
  VARIANT 12: K* denotes the modified lysine residue at X12, Ra denotes the albumin-binding moiety, Ra is "-{AEEA}2-gGlu-C(O)(CH2)16COOH
  VARIANT 23: 2-aminoisobutyric acid (Aib)
  MOD_RES 38: C-terminal amino acid residue is amidated as a primary amide
IVLSLDVPIKLKQILLEQERQRXERQQAEKNVRILERV

SEQ ID NO: 43 - protein, 38 aa, Artificial Sequence
  compound Seq_43
  VARIANT 12: K* denotes the modified lysine residue at X12, Ra denotes the albumin-binding moiety, Ra is "-{AEEA}2-gGlu-C(O)(CH2)16COOH
  MOD_RES 38: C-terminal amino acid residue is amidated as a primary amide
IVLSLDVPIKLKQILLEQAKQKKLRAQAETNVRILERV

SEQ ID NO: 44 - protein, 38 aa, Artificial Sequence
  compound Seq_44
  VARIANT 12: K* denotes the modified lysine residue at X12, Ra denotes the albumin-binding moiety, Ra is "-{AEEA}2-gGlu-C(O)(CH2)16COOH
  MOD_RES 38: C-terminal amino acid residue is amidated as a primary amide
IVLSLDVPIKLKQILLEQAKQKKERAQAETNVRILERV

SEQ ID NO: 45 - protein, 38 aa, Artificial Sequence
  compound Seq_45
  VARIANT 12: K* denotes the modified lysine residue at X12, Ra denotes the albumin-binding moiety, Ra is "-{AEEA}2-gGlu-C(O)(CH2)16COOH
  VARIANT 23: 2-aminoisobutyric acid (Aib)
  MOD_RES 38: C-terminal amino acid residue is amidated as a primary amide
IVLSLDVPIKLKQILLEQAKQKXLKAQAETNVRILERV

SEQ ID NO: 46 - protein, 38 aa, Artificial Sequence
  compound Seq_46
  VARIANT 12: K* denotes the modified lysine residue at X12, Ra denotes the albumin-binding moiety, Ra is "-{AEEA}2-gGlu-C(O)(CH2)16COOH
  VARIANT 23: 2-aminoisobutyric acid (Aib)
  MOD_RES 38: C-terminal amino acid residue is amidated as a primary amide
IVLSLDVPIKLKQILLEQAKQKXLRAQAETNVRILERV

SEQ ID NO: 47 - protein, 38 aa, Artificial Sequence
  compound Seq_47
  VARIANT 7: D-valine (v)
  VARIANT 12: K* denotes the modified lysine residue at X12, Ra denotes the albumin-binding moiety, Ra is "-{AEEA}2-gGlu-C(O)(CH2)16COOH
  VARIANT 23: 2-aminoisobutyric acid (Aib)
  MOD_RES 38: C-terminal amino acid residue is amidated as a primary amide
IVLSLDXPTKLKKKLLKQERKRXEREKAEKAARILERV

SEQ ID NO: 48 - protein, 38 aa, Artificial Sequence
  compound Seq_48
  VARIANT 12: K* denotes the modified lysine residue at X12, Ra denotes the albumin-binding moiety, Ra is "-{AEEA}2-gGlu-C(O)(CH2)16COOH
  VARIANT 23: 2-aminoisobutyric acid (Aib)
  MOD_RES 38: C-terminal amino acid residue is amidated as a primary amide
IVLSLDVPIKLKQILLEQERQRXERQQAETNVQILAQV

SEQ ID NO: 49 - protein, 38 aa, Artificial Sequence
  compound Seq_49
  VARIANT 12: K* denotes the modified lysine residue at X12, Ra denotes the albumin-binding moiety, Ra is "-{AEEA}2-gGlu-C(O)(CH2)16COOH
  VARIANT 23: 2-aminoisobutyric acid (Aib)
  MOD_RES 38: C-terminal amino acid residue is amidated as a primary amide
IVLSLDVPIKLKQILLEQERQRXERQQAETNVRILERV

SEQ ID NO: 50 - protein, 38 aa, Artificial Sequence
  compound Seq_50
  VARIANT 12: K* denotes the modified lysine residue at X12, Ra denotes the albumin-binding moiety, Ra is "-{AEEA}2-gGlu-C(O)(CH2)16COOH
  VARIANT 23: 2-aminoisobutyric acid (Aib)
  MOD_RES 38: C-terminal amino acid residue is amidated as a primary amide
IVLSLDVPTKLKQILLKQERQRXERQQAETNVRILERV

SEQ ID NO: 51 - protein, 38 aa, Artificial Sequence
  compound Seq_51
  VARIANT 12: K* denotes the modified lysine residue at X12, Ra denotes the albumin-binding moiety, Ra is "-{AEEA}2-gGlu-C(O)(CH2)16COOH
  MOD_RES 38: C-terminal amino acid residue is amidated as a primary amide
FTLSLDVPTKIKQILLKQQKQKKERQQAEKNKQLLEQI

SEQ ID NO: 52 - protein, 38 aa, Artificial Sequence
  compound Seq_52
  VARIANT 12: K* denotes the modified lysine residue at X12, Ra denotes the albumin-binding moiety, Ra is "-{AEEA}2-gGlu-C(O)(CH2)16COOH
  MOD_RES 38: C-terminal amino acid residue is amidated as a primary amide
FTLSLDVPTKIKQILLKQQKQKKERQQAEKNKQLLERV

SEQ ID NO: 53 - protein, 38 aa, Artificial Sequence
  compound Seq_53
  VARIANT 12: K* denotes the modified lysine residue at X12, Ra denotes the albumin-binding moiety, Ra is "-{AEEA}2-gGlu-C(O)(CH2)16COOH
  MOD_RES 38: C-terminal amino acid residue is amidated as a primary amide
FTLSLDVPTKIKQILLKQQKQKKERQQAETNKQLLERV

SEQ ID NO: 54 - protein, 38 aa, Artificial Sequence
  compound Seq_54
  VARIANT 12: K* denotes the modified lysine residue at X12, Ra denotes the albumin-binding moiety, Ra is "-{AEEA}2-gGlu-C(O)(CH2)16COOH
  MOD_RES 38: C-terminal amino acid residue is amidated as a primary amide
FTLSLDVPIKLKQILLKQQKQKKERQQAETNVQLLERV

SEQ ID NO: 55 - protein, 38 aa, Artificial Sequence
  compound Seq_55
  VARIANT 12: K* denotes the modified lysine residue at X12, Ra denotes the albumin-binding moiety, Ra is "-{AEEA}2-gGlu-C(O)(CH2)16COOH
  MOD_RES 38: C-terminal amino acid residue is amidated as a primary amide
FTLSLDVPTKIKQILLKQQKQKKERQKAETNVQLLERV

SEQ ID NO: 56 - protein, 38 aa, Artificial Sequence
  compound Seq_56
  VARIANT 12: K* denotes the modified lysine residue at X12, Ra denotes the albumin-binding moiety, Ra is "-{AEEA}2-gGlu-C(O)(CH2)16COOH
  MOD_RES 38: C-terminal amino acid residue is amidated as a primary amide
FTLSLDVPIGLKQILLKQQKQKKERQQAETNVQLLERV

SEQ ID NO: 57 - protein, 38 aa, Artificial Sequence
  compound Seq_57
  VARIANT 12: K* denotes the modified lysine residue at X12, Ra denotes the albumin-binding moiety, Ra is "-{AEEA}2-gGlu-C(O)(CH2)16COOH
  MOD_RES 38: C-terminal amino acid residue is amidated as a primary amide
FTLSLDVPIGLKQILLKQQKQKKERQKAETNVQLLERV

SEQ ID NO: 58 - protein, 38 aa, Artificial Sequence; identical to SEQ ID NO: 13
  compound Seq_58
  VARIANT 12: K* denotes the modified lysine residue at X12, Ra denotes the albumin-binding moiety, Ra is "-{AEEA}2-gGlu-C(O)(CH2)16COOH
  MOD_RES 38: C-terminal amino acid residue is amidated as a primary amide

SEQ ID NO: 59 - protein, 38 aa, Artificial Sequence; identical to SEQ ID NO: 51
  compound Seq_59
  VARIANT 12: K* denotes the modified lysine residue at X12, Ra denotes the albumin-binding moiety, Ra is "-{AEEA}2-gGlu-C(O)(CH2)16COOH
  MOD_RES 38: C-terminal amino acid residue is amidated as a primary amide

SEQ ID NO: 60 - protein, 38 aa, Artificial Sequence; identical to SEQ ID NO: 52
  compound Seq_60
  VARIANT 12: K* denotes the modified lysine residue at X12, Ra denotes the albumin-binding moiety, Ra is "-{AEEA}2-gGlu-C(O)(CH2)16COOH
  MOD_RES 38: C-terminal amino acid residue is amidated as a primary amide

SEQ ID NO: 61 - protein, 38 aa, Artificial Sequence; identical to SEQ ID NO: 53
  compound Seq_61
  VARIANT 12: K* denotes the modified lysine residue at X12, Ra denotes the albumin-binding moiety, Ra is "-{AEEA}2-gGlu-C(O)(CH2)16COOH
  MOD_RES 38: C-terminal amino acid residue is amidated as a primary amide

SEQ ID NO: 62 - protein, 38 aa, Artificial Sequence; identical to SEQ ID NO: 54
  compound Seq_62
  VARIANT 12: K* denotes the modified lysine residue at X12, Ra denotes the albumin-binding moiety, Ra is "-{AEEA}2-gGlu-C(O)(CH2)16COOH
  MOD_RES 38: C-terminal amino acid residue is amidated as a primary amide

SEQ ID NO: 63 - protein, 38 aa, Artificial Sequence
  compound Seq_63
  VARIANT 12: K* denotes the modified lysine residue at X12, Ra denotes the albumin-binding moiety, Ra is "-{AEEA}2-gGlu-C(O)(CH2)16COOH
  MOD_RES 38: C-terminal amino acid residue is amidated as a primary amide
FTLSLDVPIKLKQILLEQQKQKKERQQAETNVQLLERV

SEQ ID NO: 64 - protein, 38 aa, Artificial Sequence; identical to SEQ ID NO: 55
  compound Seq_64
  VARIANT 12: K* denotes the modified lysine residue at X12, Ra denotes the albumin-binding moiety, Ra is "-{AEEA}2-gGlu-C(O)(CH2)16COOH
  MOD_RES 38: C-terminal amino acid residue is amidated as a primary amide

SEQ ID NO: 65 - protein, 38 aa, Artificial Sequence; identical to SEQ ID NO: 56
  compound Seq_65
  VARIANT 12: K* denotes the modified lysine residue at X12, Ra denotes the albumin-binding moiety, Ra is "-{AEEA}2-gGlu-C(O)(CH2)16COOH
  MOD_RES 38: C-terminal amino acid residue is amidated as a primary amide

SEQ ID NO: 66 - protein, 38 aa, Artificial Sequence; identical to SEQ ID NO: 57
  compound Seq_66
  VARIANT 12: K* denotes the modified lysine residue at X12, Ra denotes the albumin-binding moiety, Ra is "-{AEEA}2-gGlu-C(O)(CH2)16COOH
  MOD_RES 38: C-terminal amino acid residue is amidated as a primary amide

SEQ ID NO: 67 - protein, 38 aa, Artificial Sequence
  compound Seq_67
  VARIANT 12: K* denotes the modified lysine residue at X12, Ra denotes the albumin-binding moiety, Ra is "-{AEEA}2-gGlu-C(O)(CH2)16COOH
  MOD_RES 38: C-terminal amino acid residue is amidated as a primary amide
IVLSLDVPIKLKQILLEQEKQKKQREQAETNKQILAQV

SEQ ID NO: 68 - protein, 38 aa, Artificial Sequence
  compound Seq_68
  VARIANT 12: K* denotes the modified lysine residue at X12, Ra denotes the albumin-binding moiety, Ra is "-{AEEA}2-gGlu-C(O)(CH2)16COOH
  MOD_RES 38: C-terminal amino acid residue is amidated as a primary amide
IVLSLDVPIKLKQILLEQERQKKQREQAETNKQILAQV

SEQ ID NO: 69 - protein, 38 aa, Artificial Sequence
  compound Seq_69
  VARIANT 12: K* denotes the modified lysine residue at X12, Ra denotes the albumin-binding moiety, Ra is "-{AEEA}2-gGlu-C(O)(CH2)16COOH
  VARIANT 14: 2-aminoisobutyric acid (Aib)
  MOD_RES 38: C-terminal amino acid residue is amidated as a primary amide
IVLSLDVPIKLKKXLLEQERQKKQREQAETNKQILAQV

SEQ ID NO: 70 - protein, 38 aa, Artificial Sequence
  compound Seq_70
  VARIANT 12: K* denotes the modified lysine residue at X12, Ra denotes the albumin-binding moiety, Ra is "-{AEEA}2-gGlu-C(O)(CH2)16COOH
  VARIANT 32: 2-aminoisobutyric acid (Aib)
  MOD_RES 38: C-terminal amino acid residue is amidated as a primary amide
IVLSLDVPIKLKQILLEQERQKKQREQAETNXQILAQV

SEQ ID NO: 71 - protein, 38 aa, Artificial Sequence
  compound Seq_71
  VARIANT 12: K* denotes the modified lysine residue at X12, Ra denotes the albumin-binding moiety, Ra is "-{AEEA}2-gGlu-C(O)(CH2)16COOH
  VARIANT 14: 2-aminoisobutyric acid (Aib)
  VARIANT 32: 2-aminoisobutyric acid (Aib)
  MOD_RES 38: C-terminal amino acid residue is amidated as a primary amide
IVLSLDVPIKLKKXLLEQERQKKQREQAETNXQILAQV

SEQ ID NO: 72 - protein, 38 aa, Artificial Sequence
  compound Seq_72
  VARIANT 12: K* denotes the modified lysine residue at X12, Ra denotes the albumin-binding moiety, Ra is "-{AEEA}2-gGlu-C(O)(CH2)16COOH
  VARIANT 32: 2-aminoisobutyric acid (Aib)
  MOD_RES 38: C-terminal amino acid residue is amidated as a primary amide
IVLSLDVPIKLKQILLEQERQKKQRQQAETNXQILAQV

SEQ ID NO: 73 - protein, 38 aa, Artificial Sequence
  compound Seq_73
  VARIANT 12: K* denotes the modified lysine residue at X12, Ra denotes the albumin-binding moiety, Ra is "-{AEEA}2-gGlu-C(O)(CH2)16COOH
  VARIANT 32: 2-aminoisobutyric acid (Aib)
  MOD_RES 38: C-terminal amino acid residue is amidated as a primary amide
IVLSLDVPIKLKQILLEQERQKKQRQKAETNXQILAQV

SEQ ID NO: 74 - protein, 38 aa, Artificial Sequence
  compound Seq_74
  VARIANT 12: K* denotes the modified lysine residue at X12, Ra denotes the albumin-binding moiety, Ra is "-{AEEA}2-gGlu-C(O)(CH2)16COOH
  VARIANT 32: 2-aminoisobutyric acid (Aib)
  MOD_RES 38: C-terminal amino acid residue is amidated as a primary amide
IVLSLDVPIKLKQILLEQERQKKQREQAETNXQILERV

SEQ ID NO: 75 - protein, 38 aa, Artificial Sequence
  compound Seq_75
  VARIANT 12: K* denotes the modified lysine residue at X12, Ra denotes the albumin-binding moiety, Ra is "-{AEEA}2-gGlu-C(O)(CH2)16COOH
  VARIANT 32: 2-aminoisobutyric acid (Aib)
  MOD_RES 38: C-terminal amino acid residue is amidated as a primary amide
IVLSLDVPIKLKQILLKQERQKKQRQQAETNXQILAQV

SEQ ID NO: 76 - protein, 38 aa, Artificial Sequence
  compound Seq_76
  VARIANT 12: K* denotes the modified lysine residue at X12, Ra denotes the albumin-binding moiety, Ra is "-{AEEA}2-gGlu-C(O)(CH2)16COOH
  VARIANT 32: 2-aminoisobutyric acid (Aib)
  MOD_RES 38: C-terminal amino acid residue is amidated as a primary amide
IVLSLDVPIGLKQILLEQERQKKQRQQAETNXQILAQV

SEQ ID NO: 77 - protein, 38 aa, Artificial Sequence
  compound Seq_77
  VARIANT 12: K* denotes the modified lysine residue at X12, Ra denotes the albumin-binding moiety, Ra is "-{AEEA}2-gGlu-C(O)(CH2)16COOH
  MOD_RES 38: C-terminal amino acid residue is amidated as a primary amide
IVLSLDVPIKLKQILLKQERQKKQRQKAETNKQILAQV

SEQ ID NO: 78 - protein, 38 aa, Artificial Sequence
  compound Seq_78
  VARIANT 12: K* denotes the modified lysine residue at X12, Ra denotes the albumin-binding moiety, Ra is "-{AEEA}2-gGlu-C(O)(CH2)16COOH
  VARIANT 32: 2-aminoisobutyric acid (Aib)
  MOD_RES 38: C-terminal amino acid residue is amidated as a primary amide
IVLSLDVPTKLKQILLEQERQKKQREQAETNXQILAQV

SEQ ID NO: 79 - protein, 38 aa, Artificial Sequence
  compound Seq_79
  VARIANT 12: K* denotes the modified lysine residue at X12, Ra denotes the albumin-binding moiety, Ra is "-{AEEA}2-gGlu-C(O)(CH2)16COOH
  VARIANT 23: 2-aminoisobutyric acid (Aib)
  MOD_RES 38: C-terminal amino acid residue is amidated as a primary amide
IVLSLDVPIKLKQILLEQEKQKXQREQAETNKQILAQV

SEQ ID NO: 80 - protein, 38 aa, Artificial Sequence; identical to SEQ ID NO: 78
  compound Seq_80
  VARIANT 12: K* denotes the modified lysine residue at X12, Ra denotes the albumin-binding moiety, Ra is "-{AEEA}2-gGlu-C(O)(CH2)16COOH
  VARIANT 32: 2-aminoisobutyric acid (Aib)
  MOD_RES 38: C-terminal amino acid residue is amidated as a primary amide

SEQ ID NO: 81 - protein, 38 aa, Artificial Sequence; identical to SEQ ID NO: 79
  compound Seq_81
  VARIANT 12: K* denotes the modified lysine residue at X12, Ra denotes the albumin-binding moiety, Ra is "-{AEEA}2-gGlu-C(O)(CH2)16COOH
  VARIANT 23: 2-aminoisobutyric acid (Aib)
  MOD_RES 38: C-terminal amino acid residue is amidated as a primary amide

SEQ ID NO: 82 - protein, 38 aa, Artificial Sequence
  compound Seq_82
  VARIANT 12: K* denotes the modified lysine residue at X12, Ra denotes the albumin-binding moiety, Ra is "-{AEEA}2-gGlu-C(O)(CH2)16COOH
  VARIANT 24: 2-aminoisobutyric acid (Aib)
  MOD_RES 38: C-terminal amino acid residue is amidated as a primary amide
IVLSLDVPTKLKQILLKQERQKKXREQAETNVRILERV

SEQ ID NO: 83 - protein, 38 aa, Artificial Sequence
  compound Seq_83
  VARIANT 7: D-valine (v)
  VARIANT 12: K* denotes the modified lysine residue at X12, Ra denotes the albumin-binding moiety, Ra is "-{AEEA}2-gGlu-C(O)(CH2)16COOH
  VARIANT 24: 2-aminoisobutyric acid (Aib)
  MOD_RES 38: C-terminal amino acid residue is amidated as a primary amide
IVLSLDXPIGLKQILLKQERQKKXREQAETNKRILERV

SEQ ID NO: 84 - protein, 38 aa, Artificial Sequence
  compound Seq_84
  VARIANT 12: K* denotes the modified lysine residue at X12, Ra denotes the albumin-binding moiety, Ra is "-{AEEA}2-gGlu-C(O)(CH2)16COOH
  MOD_RES 38: C-terminal amino acid residue is amidated as a primary amide
IVLSLDVPIKLKQKLLEQEKQKKQREQAETNKQILAQV

SEQ ID NO: 85 - protein, 38 aa, Artificial Sequence
  compound Seq_85
  VARIANT 12: K* denotes the modified lysine residue at X12, Ra denotes the albumin-binding moiety, Ra is "-{AEEA}2-gGlu-C(O)(CH2)16COOH
  MOD_RES 38: C-terminal amino acid residue is amidated as a primary amide
IVLSLDVPIKLKQILLKQERQKKQREQAETNKQILAQV

SEQ ID NO: 86 - protein, 38 aa, Artificial Sequence
  compound Seq_86
  VARIANT 12: K* denotes the modified lysine residue at X12, Ra denotes the albumin-binding moiety, Ra is "-{AEEA}2-gGlu-C(O)(CH2)16COOH
  MOD_RES 38: C-terminal amino acid residue is amidated as a primary amide
IVLSLDVPIKLKQILLKQERQKKQREQAKTNKQILAQV

SEQ ID NO: 87 - protein, 38 aa, Artificial Sequence
  compound Seq_87
  VARIANT 12: K* denotes the modified lysine residue at X12, Ra denotes the albumin-binding moiety, Ra is "-{AEEA}2-gGlu-C(O)(CH2)16COOH
  MOD_RES 38: C-terminal amino acid residue is amidated as a primary amide
IVLSLDVPIKLKQILLKQERQKKQREKAKTNKQILAQV

SEQ ID NO: 88 - protein, 38 aa, Artificial Sequence
  compound Seq_88
  VARIANT 12: K* denotes the modified lysine residue at X12, Ra denotes the albumin-binding moiety, Ra is "-{AEEA}2-gGlu-C(O)(CH2)16COOH
  VARIANT 32: 2-aminoisobutyric acid (Aib)
  MOD_RES 38: C-terminal amino acid residue is amidated as a primary amide
IVLSLDVPIKLKQILLKQERQKKQREKAKTNXQILAQV

SEQ ID NO: 89 - protein, 38 aa, Artificial Sequence
  compound Seq_89
  VARIANT 12: K* denotes the modified lysine residue at X12, Ra denotes the albumin-binding moiety, Ra is "-{AEEA}2-gGlu-C(O)(CH2)16COOH
  VARIANT 32: 2-aminoisobutyric acid (Aib)
  MOD_RES 38: C-terminal amino acid residue is amidated as a primary amide
IVLSLDVPIKLKQILLKQERQKKQREQAKTNXQILAQV

SEQ ID NO: 90 - protein, 38 aa, Artificial Sequence
  compound Seq_90
  VARIANT 12: K* denotes the modified lysine residue at X12, Ra denotes the albumin-binding moiety, Ra is "-{AEEA}2-gGlu-C(O)(CH2)16COOH
  MOD_RES 38: C-terminal amino acid residue is amidated as a primary amide
IVLSLDVPIKLKQILLKQERQKKQREKAKTNVQILAQV

SEQ ID NO: 91 - protein, 38 aa, Artificial Sequence
  compound Seq_91
  VARIANT 12: K* denotes the modified lysine residue at X12, Ra denotes the albumin-binding moiety, Ra is "-{AEEA}2-gGlu-C(O)(CH2)16COOH
  VARIANT 32: 2-aminoisobutyric acid (Aib)
  MOD_RES 38: C-terminal amino acid residue is amidated as a primary amide
IVLSLDVPIKLKQKLLKQERQKKQREKAKTNXQILAQV

SEQ ID NO: 92 - protein, 38 aa, Artificial Sequence
  compound Seq_92
  VARIANT 12: K* denotes the modified lysine residue at X12, Ra denotes the albumin-binding moiety, Ra is "-{AEEA}2-gGlu-C(O)(CH2)16COOH
  VARIANT 32: 2-aminoisobutyric acid (Aib)
  MOD_RES 38: C-terminal amino acid residue is amidated as a primary amide
IVLSLDVPIKLKQKLLEQERQKKQREQAETNXQILAQV

SEQ ID NO: 93 - protein, 38 aa, Artificial Sequence
  compound Seq_93
  VARIANT 12: K* denotes the modified lysine residue at X12, Ra denotes the albumin-binding moiety, Ra is "-{AEEA}2-gGlu-C(O)(CH2)16COOH
  MOD_RES 38: C-terminal amino acid residue is amidated as a primary amide
IVLSLDVPIKLKQKLLKQERQKKQREKAKTNVQILAQV

SEQ ID NO: 94 - protein, 38 aa, Artificial Sequence
  compound Seq_94
  VARIANT 12: K* denotes the modified lysine residue at X12, Ra denotes the albumin-binding moiety, Ra is "-{AEEA}2-gGlu-C(O)(CH2)16COOH
  MOD_RES 38: C-terminal amino acid residue is amidated as a primary amide
IVLSLDVPIKLKKILLKQERQKKEREQAETNKQILAQV

SEQ ID NO: 95 - protein, 38 aa, Artificial Sequence
  compound Seq_95
  VARIANT 12: K* denotes the modified lysine residue at X12, Ra denotes the albumin-binding moiety, Ra is "-{AEEA}2-gGlu-C(O)(CH2)16COOH
  MOD_RES 38: C-terminal amino acid residue is amidated as a primary amide
IVLSLDVPIKLKQKLLKQERQKKEREQAETNKQILAQV

SEQ ID NO: 96 - protein, 38 aa, Artificial Sequence
  compound Seq_96
  VARIANT 12: K* denotes the modified lysine residue at X12, Ra denotes the albumin-binding moiety, Ra is "-{AEEA}2-gGlu-C(O)(CH2)16COOH
  MOD_RES 38: C-terminal amino acid residue is amidated as a primary amide
IVLSLDVPIKLKQILLKQERQKKEREQAETNKQILAQV

SEQ ID NO: 97 - protein, 38 aa, Artificial Sequence
  compound Seq_97
  VARIANT 12: K* denotes the modified lysine residue at X12, Ra denotes the albumin-binding moiety, Ra is "-{AEEA}2-gGlu-C(O)(CH2)16COOH
  MOD_RES 38: C-terminal amino acid residue is amidated as a primary amide
IVLSLDVPIKLKQKLLKQERQKKQREQAETNKQILAQV

SEQ ID NO: 98 - protein, 38 aa, Artificial Sequence
  compound Seq_98
  VARIANT 12: K* denotes the modified lysine residue at X12, Ra denotes the albumin-binding moiety, Ra is "-{AEEA}2-gGlu-C(O)(CH2)16COOH
  VARIANT 24: 2-aminoisobutyric acid (Aib)
  MOD_RES 38: C-terminal amino acid residue is amidated as a primary amide
IVLSLDVPIKLKQKLLKQERQKKXREQAETNKQILAQV

SEQ ID NO: 99 - protein, 38 aa, Artificial Sequence
  compound Seq_99
  VARIANT 12: K* denotes the modified lysine residue at X12, Ra denotes the albumin-binding moiety, Ra is "-{AEEA}2-gGlu-C(O)(CH2)16COOH
  VARIANT 24: 2-aminoisobutyric acid (Aib)
  MOD_RES 38: C-terminal amino acid residue is amidated as a primary amide
IVLSLDVPIKLKKILLKQERQKKXREQAEKNKQILAQV

SEQ ID NO: 100 - protein, 38 aa, Artificial Sequence
  compound Seq_100
  VARIANT 12: K* denotes the modified lysine residue at X12, Ra denotes the albumin-binding moiety, Ra is "-{AEEA}2-gGlu-C(O)(CH2)16COOH
  VARIANT 24: 2-aminoisobutyric acid (Aib)
  VARIANT 32: 2-aminoisobutyric acid (Aib)
  MOD_RES 38: C-terminal amino acid residue is amidated as a primary amide
IVLSLDVPIKLKKILLKQERQKKXREQAETNXQILAQV

SEQ ID NO: 101 - protein, 38 aa, Artificial Sequence
  compound Seq_101
  VARIANT 12: K* denotes the modified lysine residue at X12, Ra denotes the albumin-binding moiety, Ra is "-{AEEA}2-gGlu-C(O)(CH2)16COOH
  VARIANT 24: 2-aminoisobutyric acid (Aib)
  MOD_RES 38: C-terminal amino acid residue is amidated as a primary amide
IVLSLDVPIKLKKILLKQERQKKXREQAETNKQILERV

SEQ ID NO: 102 - protein, 38 aa, Artificial Sequence
  compound Seq_102
  VARIANT 7: D-valine (v)
  VARIANT 12: K* denotes the modified lysine residue at X12, Ra denotes the albumin-binding moiety, Ra is "-{AEEA}2-gGlu-C(O)(CH2)16COOH
  MOD_RES 38: C-terminal amino acid residue is amidated as a primary amide
IVLSLDXPIKLKQILLKQERQKKQREQAETNKQILAQV

SEQ ID NO: 103 - protein, 38 aa, Artificial Sequence
  compound Seq_103
  VARIANT 12: K* denotes the modified lysine residue at X12, Ra denotes the albumin-binding moiety, Ra is "-{AEEA}2-gGlu-C(O)(CH2)16COOH
  VARIANT 23: 2-aminoisobutyric acid (Aib)
  MOD_RES 38: C-terminal amino acid residue is amidated as a primary amide
IVLSLDVPIKLKQILLEQERQKXQREQAETNKQILAQV

SEQ ID NO: 104 - protein, 38 aa, Artificial Sequence
  compound Seq_104
  VARIANT 12: K* denotes the modified lysine residue at X12, Ra denotes the albumin-binding moiety, Ra is "-{AEEA}2-gGlu-C(O)(CH2)16COOH
  VARIANT 23: 2-aminoisobutyric acid (Aib)
  MOD_RES 38: C-terminal amino acid residue is amidated as a primary amide
IVLSLDVPIKLKQILLKQERQKXQREQAETNKQILAQV

SEQ ID NO: 105 - protein, 38 aa, Artificial Sequence
  compound Seq_105
  VARIANT 12: K* denotes the modified lysine residue at X12, Ra denotes the albumin-binding moiety, Ra is "-{AEEA}2-gGlu-C(O)(CH2)16COOH
  VARIANT 23: 2-aminoisobutyric acid (Aib)
  MOD_RES 38: C-terminal amino acid residue is amidated as a primary amide
IVLSLDVPIKLKQILLEQERQKXQRQQAETNKQILAQV

SEQ ID NO: 106 - protein, 38 aa, Artificial Sequence
  compound Seq_106
  VARIANT 12: K* denotes the modified lysine residue at X12, Ra denotes the albumin-binding moiety, Ra is "-{AEEA}2-gGlu-C(O)(CH2)16COOH
  VARIANT 23: 2-aminoisobutyric acid (Aib)
  MOD_RES 38: C-terminal amino acid residue is amidated as a primary amide
IVLSLDVPIKLKQILLEQERQKXQREQAETNKQILERV

SEQ ID NO: 107 - protein, 38 aa, Artificial Sequence
  compound Seq_107
  VARIANT 12: K* denotes the modified lysine residue at X12, Ra denotes the albumin-binding moiety, Ra is "-{AEEA}2-gGlu-C(O)(CH2)16COOH
  VARIANT 23: 2-aminoisobutyric acid (Aib)
  MOD_RES 38: C-terminal amino acid residue is amidated as a primary amide
IVLSLDVPIKLKQILLKQERQKXQREQAETNKQILERV

SEQ ID NO: 108 - protein, 38 aa, Artificial Sequence
  compound Seq_108
  VARIANT 12: K* denotes the modified lysine residue at X12, Ra denotes the albumin-binding moiety, Ra is "-{AEEA}2-gGlu-C(O)(CH2)16COOH
  VARIANT 23: 2-aminoisobutyric acid (Aib)
  MOD_RES 38: C-terminal amino acid residue is amidated as a primary amide
IVLSLDVPIKLKQILLKQERQKXQRQKAETNKQILAQV

SEQ ID NO: 109 - protein, 38 aa, Artificial Sequence
  compound Seq_109
  VARIANT 12: K* denotes the modified lysine residue at X12, Ra denotes the albumin-binding moiety, Ra is "-{AEEA}2-gGlu-C(O)(CH2)16COOH
  VARIANT 23: 2-aminoisobutyric acid (Aib)
  MOD_RES 38: C-terminal amino acid residue is amidated as a primary amide
IVLSLDVPIKLKQILLKQERQKXQREKAETNKQILAQV

SEQ ID NO: 110 - protein, 38 aa, Artificial Sequence
  compound Seq_110
  VARIANT 12: K* denotes the modified lysine residue at X12, Ra denotes the albumin-binding moiety, Ra is "-{AEEA}2-gGlu-C(O)(CH2)16COOH
  VARIANT 23: 2-aminoisobutyric acid (Aib)
  MOD_RES 38: C-terminal amino acid residue is amidated as a primary amide
IVLSLDVPIKLKQILLKQERQKXQRQQAETNKQILAQV

SEQ ID NO: 111 - protein, 38 aa, Artificial Sequence
  compound Seq_111
  VARIANT 12: K* denotes the modified lysine residue at X12, Ra denotes the albumin-binding moiety, Ra is "-{AEEA}2-gGlu-C(O)(CH2)16COOH
  MOD_RES 38: C-terminal amino acid residue is amidated as a primary amide
IVLSLDVPIKLKQILLKQERQKKQREQAETNKQILEQV

SEQ ID NO: 112 - protein, 38 aa, Artificial Sequence
  compound Seq_112
  VARIANT 12: K* denotes the modified lysine residue at X12, Ra denotes the albumin-binding moiety, Ra is "-{AEEA}2-gGlu-C(O)(CH2)16COOH
  MOD_RES 38: C-terminal amino acid residue is amidated as a primary amide
IVLSLDVPIKLKQILLKQERQKKQREKAETNKQILAQV

SEQ ID NO: 113 - protein, 38 aa, Artificial Sequence
  compound Seq_113
  VARIANT 12: K* denotes the modified lysine residue at X12, Ra denotes the albumin-binding moiety, Ra is "-{AEEA}2-gGlu-C(O)(CH2)16COOH
  MOD_RES 38: C-terminal amino acid residue is amidated as a primary amide
IVLSLDVPIKLKQILLKQERQKKQRQQAETNKQILAQV

SEQ ID NO: 114 - protein, 38 aa, Artificial Sequence
  compound Seq_114
  VARIANT 12: K* denotes the modified lysine residue at X12, Ra denotes the albumin-binding moiety, Ra is "-{AEEA}2-gGlu-C(O)(CH2)16COOH
  VARIANT 23: 2-aminoisobutyric acid (Aib)
  MOD_RES 38: C-terminal amino acid residue is amidated as a primary amide
IVLSLDVPIKLKQILLEQARQKXQRAQAETNKRILERV

SEQ ID NO: 115 - protein, 38 aa, Artificial Sequence
  compound Seq_115
  VARIANT 12: K* denotes the modified lysine residue at X12, Ra denotes the albumin-binding moiety, Ra is "-{AEEA}2-gGlu-C(O)(CH2)16COOH
  VARIANT 23: 2-aminoisobutyric acid (Aib)
  MOD_RES 38: C-terminal amino acid residue is amidated as a primary amide
IVLSLDVPIKLKQILLKQERQKXQREQAEKNKQILERV

SEQ ID NO: 116 - protein, 38 aa, Artificial Sequence
  compound Seq_116
  VARIANT 12: K* denotes the modified lysine residue at X12, Ra denotes the albumin-binding moiety, Ra is "-{AEEA}2-gGlu-C(O)(CH2)16COOH
  VARIANT 23: 2-aminoisobutyric acid (Aib)
  MOD_RES 38: C-terminal amino acid residue is amidated as a primary amide
IVLSLDVPIKLKQILLKQERQKXQREKAEKNKQILAQV

SEQ ID NO: 117 - protein, 38 aa, Artificial Sequence
  compound Seq_117
  VARIANT 12: K* denotes the modified lysine residue at X12, Ra denotes the albumin-binding moiety, Ra is "-{AEEA}2-gGlu-C(O)(CH2)16COOH
  VARIANT 23: 2-aminoisobutyric acid (Aib)
  MOD_RES 38: C-terminal amino acid residue is amidated as a primary amide
IVLSLDVPIKLKQILLKQERQKXQRQQAEKNKQILAQV

SEQ ID NO: 118 - protein, 38 aa, Artificial Sequence
  compound Seq_118
  VARIANT 7: D-valine (v)
  VARIANT 12: K* denotes the modified lysine residue at X12, Ra denotes the albumin-binding moiety, Ra is "-{AEEA}2-gGlu-C(O)(CH2)16COOH
  VARIANT 23: 2-aminoisobutyric acid (Aib)
  MOD_RES 38: C-terminal amino acid residue is amidated as a primary amide
IVLSLDXPIKLKQILLKQERQKXQRQKAEKNKQILAQV

SEQ ID NO: 119 - protein, 38 aa, Artificial Sequence
  compound Seq_119
  VARIANT 12: K* denotes the modified lysine residue at X12, Ra denotes the albumin-binding moiety, Ra is "-{AEEA}2-gGlu-C(O)(CH2)16COOH
  VARIANT 24: 2-aminoisobutyric acid (Aib)
  MOD_RES 38: C-terminal amino acid residue is amidated as a primary amide
IVLSLDVPIKLKQILLKQERQKKXRQKAEKNKQILAQV

SEQ ID NO: 120 - protein, 38 aa, Artificial Sequence
  compound Seq_120
  VARIANT 12: K* denotes the modified lysine residue at X12, Ra denotes the albumin-binding moiety, Ra is "-{AEEA}2-gGlu-C(O)(CH2)16COOH
  MOD_RES 38: C-terminal amino acid residue is amidated as a primary amide
IVLSLDVPIKLKQILLKQERQKKQREQAEKNKQILEQV

SEQ ID NO: 121 - protein, 38 aa, Artificial Sequence
  compound Seq_121
  VARIANT 12: K* denotes the modified lysine residue at X12, Ra denotes the albumin-binding moiety, Ra is "-{AEEA}2-gGlu-C(O)(CH2)16COOH
  MOD_RES 38: C-terminal amino acid residue is amidated as a primary amide
IVLSLDVPIKLKQILLKQERQKKQREKAEKNKQILAQV

SEQ ID NO: 122 - protein, 38 aa, Artificial Sequence
  compound Seq_122
  VARIANT 12: K* denotes the modified lysine residue at X12, Ra denotes the albumin-binding moiety, Ra is "-{AEEA}2-gGlu-C(O)(CH2)16COOH
  MOD_RES 38: C-terminal amino acid residue is amidated as a primary amide
IVLSLDVPIKLKQILLKQERQKKQRQQAEKNKQILAQV

SEQ ID NO: 123 - protein, 38 aa, Artificial Sequence
  compound Seq_123
  VARIANT 12: K* denotes the modified lysine residue at X12, Ra denotes the albumin-binding moiety, Ra is "-{AEEA}2-gGlu-C(O)(CH2)16COOH
  VARIANT 23: 2-aminoisobutyric acid (Aib)
  MOD_RES 38: C-terminal amino acid residue is amidated as a primary amide
IVLSLDVPIKLKQILLEQARQKXQRAQAEKNKRILERV

SEQ ID NO: 124 - protein, 38 aa, Artificial Sequence
  compound Seq_124
  VARIANT 12: K* denotes the modified lysine residue at X12, Ra denotes the albumin-binding moiety, Ra is "-{AEEA}2-gGlu-C(O)(CH2)16COOH
  VARIANT 23: 2-aminoisobutyric acid (Aib)
  MOD_RES 38: C-terminal amino acid residue is amidated as a primary amide
IVLSLDVPIKLKQILLKQARQKXQRAQAEKNKRILERV

SEQ ID NO: 125 - protein, 38 aa, Artificial Sequence
  compound Seq_125
  VARIANT 12: K* denotes the modified lysine residue at X12, Ra denotes the albumin-binding moiety, Ra is "-{AEEA}2-gGlu-C(O)(CH2)16COOH
  VARIANT 23: 2-aminoisobutyric acid (Aib)
  MOD_RES 38: C-terminal amino acid residue is amidated as a primary amide
IVLSLDVPIKLKQILLEQARQKXQREQAEKNKRILERV

SEQ ID NO: 126 - protein, 38 aa, Artificial Sequence
  compound Seq_126
  VARIANT 7: D-valine (v)
  VARIANT 12: K* denotes the modified lysine residue at X12, Ra denotes the albumin-binding moiety, Ra is "-{AEEA}2-gGlu-C(O)(CH2)16COOH
  VARIANT 23: 2-aminoisobutyric acid (Aib)
  MOD_RES 38: C-terminal amino acid residue is amidated as a primary amide
IVLSLDXPIKLKQILLEQAKQKXQRAQAEKNKRILERV

SEQ ID NO: 127 - protein, 38 aa, Artificial Sequence
  compound Seq_127
  VARIANT 7: D-valine (v)
  VARIANT 12: K* denotes the modified lysine residue at X12, Ra denotes the albumin-binding moiety, Ra is "-{AEEA}2-gGlu-C(O)(CH2)16COOH
  VARIANT 23: 2-aminoisobutyric acid (Aib)
  MOD_RES 38: C-terminal amino acid residue is amidated as a primary amide
IVLSLDXPIKLKQILLEQAKQKXQREQAEKNKRILERV

SEQ ID NO: 128 - protein, 38 aa, Artificial Sequence
  compound Seq_128
  VARIANT 7: D-valine (v)
  VARIANT 12: K* denotes the modified lysine residue at X12, Ra denotes the albumin-binding moiety, Ra is "-{AEEA}2-gGlu-C(O)(CH2)16COOH
  VARIANT 23: 2-aminoisobutyric acid (Aib)
  MOD_RES 38: C-terminal amino acid residue is amidated as a primary amide
IVLSLDXPIKLKQILLKQARQKXQREQAEKNKRILERV

SEQ ID NO: 129 - protein, 38 aa, Artificial Sequence
  compound Seq_129
  VARIANT 7: D-valine (v)
  VARIANT 12: K* denotes the modified lysine residue at X12, Ra denotes the albumin-binding moiety, Ra is "-{AEEA}2-gGlu-C(O)(CH2)16COOH
  VARIANT 23: 2-aminoisobutyric acid (Aib)
  MOD_RES 38: C-terminal amino acid residue is amidated as a primary amide
IVLSLDXPIKLKQILLEQERQKXQREQAEKNKQILAQV

SEQ ID NO: 130 - protein, 38 aa, Artificial Sequence
  compound Seq_130
  VARIANT 7: D-valine (v)
  VARIANT 12: K* denotes the modified lysine residue at X12, Ra denotes the albumin-binding moiety, Ra is "-{AEEA}2-gGlu-C(O)(CH2)16COOH
  VARIANT 23: 2-aminoisobutyric acid (Aib)
  MOD_RES 38: C-terminal amino acid residue is amidated as a primary amide
IVLSLDXPIKLKQILLKQERQKXQREQAEKNKQILAQV

SEQ ID NO: 131 - protein, 38 aa, Artificial Sequence
  compound Seq_131
  VARIANT 7: D-valine (v)
  VARIANT 12: K* denotes the modified lysine residue at X12, Ra denotes the albumin-binding moiety, Ra is "-{AEEA}2-gGlu-C(O)(CH2)16COOH
  VARIANT 23: 2-aminoisobutyric acid (Aib)
  MOD_RES 38: C-terminal amino acid residue is amidated as a primary amide
IVLSLDXPIKLKQILLEQERQKXQRQQAEKNKQILAQV

SEQ ID NO: 132 - protein, 38 aa, Artificial Sequence
  compound Seq_132
  VARIANT 7: D-valine (v)
  VARIANT 12: K* denotes the modified lysine residue at X12, Ra denotes the albumin-binding moiety, Ra is "-{AEEA}2-gGlu-C(O)(CH2)16COOH
  VARIANT 23: 2-aminoisobutyric acid (Aib)
  MOD_RES 38: C-terminal amino acid residue is amidated as a primary amide
IVLSLDXPIKLKQILLEQERQKXQREQAEKNKQILERV

SEQ ID NO: 133 - protein, 38 aa, Artificial Sequence
  compound Seq_133
  VARIANT 7: D-valine (v)
  VARIANT 12: K* denotes the modified lysine residue at X12, Ra denotes the albumin-binding moiety, Ra is "-{AEEA}2-gGlu-C(O)(CH2)16COOH
  VARIANT 23: 2-aminoisobutyric acid (Aib)
  MOD_RES 38: C-terminal amino acid residue is amidated as a primary amide
IVLSLDXPIKLKQILLKQERQKXQREQAEKNKQILERV

SEQ ID NO: 134 - protein, 38 aa, Artificial Sequence
  compound Seq_134
  VARIANT 7: D-valine (v)
  VARIANT 12: K* denotes the modified lysine residue at X12, Ra denotes the albumin-binding moiety, Ra is "-{AEEA}2-gGlu-C(O)(CH2)16COOH
  VARIANT 23: 2-aminoisobutyric acid (Aib)
  MOD_RES 38: C-terminal amino acid residue is amidated as a primary amide
IVLSLDXPIKLKQILLKQERQKXQREKAEKNKQILAQV

SEQ ID NO: 135 - protein, 38 aa, Artificial Sequence
  compound Seq_135
  VARIANT 7: D-valine (v)
  VARIANT 12: K* denotes the modified lysine residue at X12, Ra denotes the albumin-binding moiety, Ra is "-{AEEA}2-gGlu-C(O)(CH2)16COOH
  VARIANT 23: 2-aminoisobutyric acid (Aib)
  MOD_RES 38: C-terminal amino acid residue is amidated as a primary amide
IVLSLDXPIKLKQILLKQERQKXQRQQAEKNKQILAQV

SEQ ID NO: 136 - protein, 38 aa, Artificial Sequence
  compound Seq_136
  VARIANT 7: D-valine (v)
  VARIANT 12: K* denotes the modified lysine residue at X12, Ra denotes the albumin-binding moiety, Ra is "-{AEEA}2-gGlu-C(O)(CH2)16COOH
  VARIANT 24: 2-aminoisobutyric acid (Aib)
  MOD_RES 38: C-terminal amino acid residue is amidated as a primary amide
IVLSLDXPIKLKQILLKQERQKKXRQKAEKNKQILAQV

SEQ ID NO: 137 - protein, 38 aa, Artificial Sequence
  compound Seq_137
  VARIANT 7: D-valine (v)
  VARIANT 12: K* denotes the modified lysine residue at X12, Ra denotes the albumin-binding moiety, Ra is "-{AEEA}2-gGlu-C(O)(CH2)16COOH
  MOD_RES 38: C-terminal amino acid residue is amidated as a primary amide
IVLSLDXPIKLKQILLKQERQKKQREQAEKNKQILEQV

SEQ ID NO: 138 - protein, 38 aa, Artificial Sequence
  compound Seq_138
  VARIANT 7: D-valine (v)
  VARIANT 12: K* denotes the modified lysine residue at X12, Ra denotes the albumin-binding moiety, Ra is "-{AEEA}2-gGlu-C(O)(CH2)16COOH
  MOD_RES 38: C-terminal amino acid residue is amidated as a primary amide
IVLSLDXPIKLKQILLKQERQKKQREKAEKNKQILAQV

SEQ ID NO: 139 - protein, 38 aa, Artificial Sequence
  compound Seq_139
  VARIANT 7: D-valine (v)
  VARIANT 12: K* denotes the modified lysine residue at X12, Ra denotes the albumin-binding moiety, Ra is "-{AEEA}2-gGlu-C(O)(CH2)16COOH
  MOD_RES 38: C-terminal amino acid residue is amidated as a primary amide
IVLSLDXPIKLKQILLKQERQKKQRQQAEKNKQILAQV

SEQ ID NO: 140 - protein, 38 aa, Artificial Sequence
  compound Seq_140
  VARIANT 7: D-valine (v)
  VARIANT 12: K* denotes the modified lysine residue at X12, Ra denotes the albumin-binding moiety, Ra is "-{AEEA}2-gGlu-C(O)(CH2)16COOH
  VARIANT 23: 2-aminoisobutyric acid (Aib)
  MOD_RES 38: C-terminal amino acid residue is amidated as a primary amide
IVLSLDXPIKLKQILLEQARQKXQRAQAEKNKRILERV

SEQ ID NO: 141 - protein, 38 aa, Artificial Sequence
  compound Seq_141
  VARIANT 7: D-valine (v)
  VARIANT 12: K* denotes the modified lysine residue at X12, Ra denotes the albumin-binding moiety, Ra is "-{AEEA}2-gGlu-C(O)(CH2)16COOH
  VARIANT 23: 2-aminoisobutyric acid (Aib)
  MOD_RES 38: C-terminal amino acid residue is amidated as a primary amide
IVLSLDXPIKLKQILLKQARQKXQRAQAEKNKRILERV

SEQ ID NO: 142 - protein, 38 aa, Artificial Sequence
  compound Seq_142
  VARIANT 7: D-valine (v)
  VARIANT 12: K* denotes the modified lysine residue at X12, Ra denotes the albumin-binding moiety, Ra is "-{AEEA}2-gGlu-C(O)(CH2)16COOH
  VARIANT 23: 2-aminoisobutyric acid (Aib)
  MOD_RES 38: C-terminal amino acid residue is amidated as a primary amide
IVLSLDXPIKLKQILLEQARQKXQREQAEKNKRILERV

SEQ ID NO: 143 - protein, 38 aa, Artificial Sequence
  compound Seq_143
  VARIANT 12: K* denotes the modified lysine residue at X12, Ra denotes the albumin-binding moiety, Ra is "-{AEEA}2-gGlu-C(O)(CH2)16COOH
  MOD_RES 38: C-terminal amino acid residue is amidated as a primary amide
FTLSLDVPTKIKQILLKQEKQKKQRQKAKTNKQILERV

SEQ ID NO: 144 - protein, 38 aa, Artificial Sequence
  compound Seq_144
  VARIANT 12: K* denotes the modified lysine residue at X12, Ra denotes the albumin-binding moiety, Ra is "-{AEEA}2-gGlu-C(O)(CH2)16COOH
  MOD_RES 38: C-terminal amino acid residue is amidated as a primary amide
FTLSLDVPTKIKQILLKQERQKKQRQKAKTNKQILERV

SEQ ID NO: 145 - protein, 38 aa, Artificial Sequence
  compound Seq_145
  VARIANT 12: K* denotes the modified lysine residue at X12, Ra denotes the albumin-binding moiety, Ra is "-{AEEA}2-gGlu-C(O)(CH2)16COOH
  MOD_RES 38: C-terminal amino acid residue is amidated as a primary amide
FTLSLDVPTKIKQILLKQERQKKQRQKAKKNKQILERV

SEQ ID NO: 146 - protein, 38 aa, Artificial Sequence
  compound Seq_146
  VARIANT 12: K* denotes the modified lysine residue at X12, Ra denotes the albumin-binding moiety, Ra is "-{AEEA}2-gGlu-C(O)(CH2)16COOH
  MOD_RES 38: C-terminal amino acid residue is amidated as a primary amide
FTLSLDVPIKLKQILLKQERQKKQRQKAKKNKQILERV

SEQ ID NO: 147 - protein, 38 aa, Artificial Sequence
  compound Seq_147
  VARIANT 7: D-valine (v)
  VARIANT 12: K* denotes the modified lysine residue at X12, Ra denotes the albumin-binding moiety, Ra is "-{AEEA}2-gGlu-C(O)(CH2)16COOH
  VARIANT 24: 2-aminoisobutyric acid (Aib)
  MOD_RES 38: C-terminal amino acid residue is amidated as a primary amide
IVLSLDXPIGLKQILLKQERQKKXREQAETNKQILAQV

SEQ ID NO: 148 - protein, 38 aa, Artificial Sequence
  compound Seq_148
  VARIANT 12: K* denotes the modified lysine residue at X12, Ra denotes the albumin-binding moiety, Ra is "-{AEEA}2-gGlu-C(O)(CH2)16COOH
  VARIANT 24: 2-aminoisobutyric acid (Aib)
  MOD_RES 38: C-terminal amino acid residue is amidated as a primary amide
IVLSLDVPIGLKQILLKQERQKKXREQAETNKRILERV

SEQ ID NO: 149 - protein, 38 aa, Artificial Sequence
  compound Seq_149
  VARIANT 7: D-valine (v)
  VARIANT 12: K* denotes the modified lysine residue at X12, Ra denotes the albumin-binding moiety, Ra is "-{AEEA}2-gGlu-C(O)(CH2)16COOH
  VARIANT 24: 2-aminoisobutyric acid (Aib)
  MOD_RES 38: C-terminal amino acid residue is amidated as a primary amide
IVLSLDXPIKLKQILLKQERQKKXREQAETNKRILERV

SEQ ID NO: 150 - protein, 38 aa, Artificial Sequence
  compound Seq_150
  VARIANT 7: D-valine (v)
  VARIANT 12: K* denotes the modified lysine residue at X12, Ra denotes the albumin-binding moiety, Ra is "-{AEEA}2-gGlu-C(O)(CH2)16COOH
  VARIANT 24: 2-aminoisobutyric acid (Aib)
  MOD_RES 38: C-terminal amino acid residue is amidated as a primary amide
IVLSLDXPIGLKQILLKQERQKKXRQQAETNKRILERV

SEQ ID NO: 151 - protein, 38 aa, Artificial Sequence
  compound Seq_151
  VARIANT 7: D-valine (v)
  VARIANT 12: K* denotes the modified lysine residue at X12, Ra denotes the albumin-binding moiety, Ra is "-{AEEA}2-gGlu-C(O)(CH2)16COOH
  VARIANT 24: 2-aminoisobutyric acid (Aib)
  MOD_RES 38: C-terminal amino acid residue is amidated as a primary amide
IVLSLDXPIGLKQILLKQERQKKXREQAEKNKRILERV

SEQ ID NO: 152 - protein, 38 aa, Artificial Sequence
  compound Seq_152
  VARIANT 12: K* denotes the modified lysine residue at X12, Ra denotes the albumin-binding moiety, Ra is "-{AEEA}2-gGlu-C(O)(CH2)16COOH
  VARIANT 24: 2-aminoisobutyric acid (Aib)
  MOD_RES 38: C-terminal amino acid residue is amidated as a primary amide
IVLSLDVPIKLKQILLKQERQKKXREQAETNKRILERV

SEQ ID NO: 153 - protein, 38 aa, Artificial Sequence; identical to SEQ ID NO: 1
  MOD_RES 1: Acetylation
  compound Seq_153
  VARIANT 12: K* denotes the modified lysine residue at X12, Ra denotes the albumin-binding moiety, Ra is "-{AEEA}2-gGlu-C(O)(CH2)16COOH
  MOD_RES 38: C-terminal amino acid residue is amidated as a primary amide

SEQ ID NO: 154 - protein, 38 aa, Artificial Sequence
  compound Seq_154
  VARIANT 12: K* denotes the modified lysine residue at X12, Ra denotes the albumin-binding moiety, Ra is "-{AEEA}2-gGlu-C(O)(CH2)16COOH
  MOD_RES 38: C-terminal amino acid residue is amidated as a primary amide
IVLSLDVPIGLKQILLEQEKQEKEKQQAETNKRILERV

SEQ ID NO: 155 - protein, 38 aa, Artificial Sequence
  compound Seq_155
  VARIANT 12: K* denotes the modified lysine residue at X12, Ra denotes the albumin-binding moiety, Ra is "-{AEEA}2-gGlu-C(O)(CH2)16COOH
  MOD_RES 38: C-terminal amino acid residue is amidated as a primary amide
IVLSLDVPIGLKQILLEQEKQEKEKQQAEKNKRILERV

SEQ ID NO: 156 - protein, 38 aa, Artificial Sequence
  compound Seq_156
  VARIANT 12: K* denotes the modified lysine residue at X12, Ra denotes the albumin-binding moiety, Ra is "-{AEEA}2-gGlu-C(O)(CH2)16COOH
  VARIANT 24: 2-aminoisobutyric acid (Aib)
  MOD_RES 38: C-terminal amino acid residue is amidated as a primary amide
IVLSLDVPIGLKQILLKQERQKKXREQAETNAQILAQV

SEQ ID NO: 157 - protein, 38 aa, Artificial Sequence
  MOD_RES 1: Acetylation
  compound Seq_157
  VARIANT 7: D-valine (v)
  VARIANT 12: K* denotes the modified lysine residue at X12, Ra denotes the albumin-binding moiety, Ra is "-{AEEA}2-gGlu-C(O)(CH2)16COOH
  VARIANT 23: 2-aminoisobutyric acid (Aib)
  MOD_RES 38: C-terminal amino acid residue is amidated as a primary amide
IVLSLDXPIKLKQILLEQARQKXQREQAEKNKQILEQV

SEQ ID NO: 158 - protein, 38 aa, Artificial Sequence
  MOD_RES 1: Acetylation
  compound Seq_158
  VARIANT 7: D-valine (v)
  VARIANT 12: K* denotes the modified lysine residue at X12, Ra denotes the albumin-binding moiety, Ra is "-{AEEA}2-gGlu-C(O)(CH2)16COOH
  VARIANT 23: 2-aminoisobutyric acid (Aib)
  MOD_RES 38: C-terminal amino acid residue is amidated as a primary amide
IVLSLDXPIKLKQILLEQERQKXQREQAEKNKQILEQV

SEQ ID NO: 159 - protein, 38 aa, Artificial Sequence
  MOD_RES 1: Acetylation
  compound Seq_159
  VARIANT 7: D-valine (v)
  VARIANT 12: K* denotes the modified lysine residue at X12, Ra denotes the albumin-binding moiety, Ra is "-{AEEA}2-gGlu-C(O)(CH2)16COOH
  VARIANT 23: 2-aminoisobutyric acid (Aib)
  MOD_RES 38: C-terminal amino acid residue is amidated as a primary amide
IVLSLDXPIKLKQILLEQERQEXQREQAEKNKQILEQV

SEQ ID NO: 160 - protein, 38 aa, Artificial Sequence
  MOD_RES 1: Acetylation
  compound Seq_160
  VARIANT 7: D-valine (v)
  VARIANT 12: K* denotes the modified lysine residue at X12, Ra denotes the albumin-binding moiety, Ra is "-{AEEA}2-gGlu-C(O)(CH2)16COOH
  VARIANT 23: 2-aminoisobutyric acid (Aib)
  MOD_RES 38: C-terminal amino acid residue is amidated as a primary amide
IVLSLDXPIKLKQILLEQERQEXEREQAETNKQILEQV

SEQ ID NO: 161 - protein, 38 aa, Artificial Sequence
  MOD_RES 1: Acetylation
  compound Seq_161
  VARIANT 7: D-valine (v)
  VARIANT 12: K* denotes the modified lysine residue at X12, Ra denotes the albumin-binding moiety, Ra is "-{AEEA}2-gGlu-C(O)(CH2)16COOH
  VARIANT 23: 2-aminoisobutyric acid (Aib)
  MOD_RES 38: C-terminal amino acid residue is amidated as a primary amide
IVLSLDXPIKLKQILLEQERQEXEREQAEKNEQILEQV

SEQ ID NO: 162 - protein, 38 aa, Artificial Sequence
  MOD_RES 1: Acetylation
  compound Seq_162
  VARIANT 7: D-valine (v)
  VARIANT 12: K* denotes the modified lysine residue at X12, Ra denotes the albumin-binding moiety, Ra is "-{AEEA}2-gGlu-C(O)(CH2)16COOH
  VARIANT 23: 2-aminoisobutyric acid (Aib)
  MOD_RES 38: C-terminal amino acid residue is amidated as a primary amide
IVLSLDXPIELKQILLEQERQKXQREQAEKNKQILEQV

SEQ ID NO: 163 - protein, 38 aa, Artificial Sequence
  MOD_RES 1: Acetylation
  compound Seq_163
  VARIANT 7: D-valine (v)
  VARIANT 12: K* denotes the modified lysine residue at X12, Ra denotes the albumin-binding moiety, Ra is "-{AEEA}2-gGlu-C(O)(CH2)16COOH
  VARIANT 23: 2-aminoisobutyric acid (Aib)
  MOD_RES 38: C-terminal amino acid residue is amidated as a primary amide
IVLSLDXPIHLKQILLEQERQKXQREQAEKNKQILEQV

SEQ ID NO: 164 - protein, 38 aa, Artificial Sequence
  MOD_RES 1: Acetylation
  compound Seq_164
  VARIANT 7: D-valine (v)
  VARIANT 12: K* denotes the modified lysine residue at X12, Ra denotes the albumin-binding moiety, Ra is "-{AEEA}2-gGlu-C(O)(CH2)16COOH
  VARIANT 23: 2-aminoisobutyric acid (Aib)
  MOD_RES 38: C-terminal amino acid residue is amidated as a primary amide
IVLSLDXPIGLKQILLEQERQKXQREQAEKNKQILEQV

SEQ ID NO: 165 - protein, 38 aa, Artificial Sequence
  MOD_RES 1: Acetylation
  compound Seq_165
  VARIANT 7: D-valine (v)
  VARIANT 12: K* denotes the modified lysine residue at X12, Ra denotes the albumin-binding moiety, Ra is "-{AEEA}2-gGlu-C(O)(CH2)16COOH
  VARIANT 23: 2-aminoisobutyric acid (Aib)
  MOD_RES 38: C-terminal amino acid residue is amidated as a primary amide
IVLSLDXPIKLKQILLEQARQKXQREQAEKNEQILEQV

SEQ ID NO: 166 - protein, 38 aa, Artificial Sequence
  MOD_RES 1: Acetylation
  compound Seq_166
  VARIANT 7: D-valine (v)
  VARIANT 12: K* denotes the modified lysine residue at X12, Ra denotes the albumin-binding moiety, Ra is "-{AEEA}2-gGlu-C(O)(CH2)16COOH
  VARIANT 23: 2-aminoisobutyric acid (Aib)
  MOD_RES 38: C-terminal amino acid residue is amidated as a primary amide
IVLSLDXPIKLKQILLEQERQKXQREQAEKNEQILEQV

SEQ ID NO: 167 - protein, 38 aa, Artificial Sequence
  MOD_RES 1: Acetylation
  compound Seq_167
  VARIANT 7: D-valine (v)
  VARIANT 12: K* denotes the modified lysine residue at X12, Ra denotes the albumin-binding moiety, Ra is "-{AEEA}2-gGlu-C(O)(CH2)16COOH
  VARIANT 23: 2-aminoisobutyric acid (Aib)
  MOD_RES 38: C-terminal amino acid residue is amidated as a primary amide
IVLSLDXPIGLKQILLEQERQKXQREQAEKNEQILEQV

SEQ ID NO: 168 - protein, 38 aa, Artificial Sequence
  MOD_RES 1: Acetylation
  compound Seq_168
  VARIANT 7: D-valine (v)
  VARIANT 12: K* denotes the modified lysine residue at X12, Ra denotes the albumin-binding moiety, Ra is "-{AEEA}2-gGlu-C(O)(CH2)16COOH
  VARIANT 23: 2-aminoisobutyric acid (Aib)
  MOD_RES 38: C-terminal amino acid residue is amidated as a primary amide
IVLSLDXPIELKQILLEQERQKXQREQAEKNEQILEQV

SEQ ID NO: 169 - protein, 38 aa, Artificial Sequence
  MOD_RES 1: Acetylation
  compound Seq_169
  VARIANT 7: D-valine (v)
  VARIANT 12: K* denotes the modified lysine residue at X12, Ra denotes the albumin-binding moiety, Ra is "-{AEEA}2-gGlu-C(O)(CH2)16COOH
  VARIANT 23: 2-aminoisobutyric acid (Aib)
  MOD_RES 38: C-terminal amino acid residue is amidated as a primary amide
IVLSLDXPIKLKQILLEQERQEXQREQAEKNEQILEQV

SEQ ID NO: 170 - protein, 38 aa, Artificial Sequence
  MOD_RES 1: Acetylation
  compound Seq_170
  VARIANT 7: D-valine (v)
  VARIANT 12: K* denotes the modified lysine residue at X12, Ra denotes the albumin-binding moiety, Ra is "-{AEEA}2-gGlu-C(O)(CH2)16COOH
  VARIANT 23: 2-aminoisobutyric acid (Aib)
  MOD_RES 38: C-terminal amino acid residue is amidated as a primary amide
IVLSLDXPIELKQILLEQERQEXQREQAEKNEQILEQV

SEQ ID NO: 171 - protein, 38 aa, Artificial Sequence; identical to SEQ ID NO: 130
  compound Seq_171
  VARIANT 7: D-valine (v)
  VARIANT 12: K* denotes the modified lysine residue at X12, Ra denotes the albumin-binding moiety, Ra is "-{AEEA}2-{gGlu}2-C(O)(CH2)16COOH
  VARIANT 23: 2-aminoisobutyric acid (Aib)
  MOD_RES 38: C-terminal amino acid residue is amidated as a primary amide

SEQ ID NO: 172 - protein, 38 aa, Artificial Sequence; identical to SEQ ID NO: 130
  compound Seq_172
  VARIANT 7: D-valine (v)
  VARIANT 12: K* denotes the modified lysine residue at X12, Ra denotes the albumin-binding moiety, Ra is "-{AEEA}2-{gGlu}2-C(O)(CH2)16COOH
  VARIANT 23: 2-aminoisobutyric acid (Aib)
  MOD_RES 38: C-terminal amino acid residue is amidated as a primary amide

SEQ ID NO: 173 - protein, 38 aa, Artificial Sequence; identical to SEQ ID NO: 130
  compound Seq_173
  VARIANT 7: D-valine (v)
  VARIANT 12: K* denotes the modified lysine residue at X12, Ra denotes the albumin-binding moiety, Ra is "-{AEEA}2-gGlu-C(O)(CH2)18COOH
  VARIANT 23: 2-aminoisobutyric acid (Aib)
  MOD_RES 38: C-terminal amino acid residue is amidated as a primary amide

SEQ ID NO: 174 - protein, 38 aa, Artificial Sequence; identical to SEQ ID NO: 141
  compound Seq_174
  VARIANT 7: D-valine (v)
  VARIANT 12: K* denotes the modified lysine residue at X12, Ra denotes the albumin-binding moiety, Ra is "-{AEEA}2-{gGlu}2-C(O)(CH2)16COOH
  VARIANT 23: 2-aminoisobutyric acid (Aib)
  MOD_RES 38: C-terminal amino acid residue is amidated as a primary amide

SEQ ID NO: 175 - protein, 38 aa, Artificial Sequence; identical to SEQ ID NO: 141
  compound Seq_175
  VARIANT 7: D-valine (v)
  VARIANT 12: K* denotes the modified lysine residue at X12, Ra denotes the albumin-binding moiety, Ra is "-{AEEA}2-gGlu-C(O)(CH2)18COOH
  VARIANT 23: 2-aminoisobutyric acid (Aib)
  MOD_RES 38: C-terminal amino acid residue is amidated as a primary amide

SEQ ID NO: 176 - protein, 38 aa, Artificial Sequence; identical to SEQ ID NO: 139
  compound Seq_176
  VARIANT 7: D-valine (v)
  VARIANT 12: K* denotes the modified lysine residue at X12, Ra denotes the albumin-binding moiety, Ra is "-{AEEA}2-{gGlu}2-C(O)(CH2)16COOH
  MOD_RES 38: C-terminal amino acid residue is amidated as a primary amide

SEQ ID NO: 177 - protein, 38 aa, Artificial Sequence; identical to SEQ ID NO: 139
  compound Seq_177
  VARIANT 7: D-valine (v)
  VARIANT 12: K* denotes the modified lysine residue at X12, Ra denotes the albumin-binding moiety, Ra is "-{AEEA}2-{gGlu}2-C(O)(CH2)16COOH
  MOD_RES 38: C-terminal amino acid residue is amidated as a primary amide

SEQ ID NO: 178 - protein, 38 aa, Artificial Sequence; identical to SEQ ID NO: 139
  compound Seq_178
  VARIANT 7: D-valine (v)
  VARIANT 12: K* denotes the modified lysine residue at X12, Ra denotes the albumin-binding moiety, Ra is "-{AEEA}2-gGlu-C(O)(CH2)18COOH
  MOD_RES 38: C-terminal amino acid residue is amidated as a primary amide

SEQ ID NO: 179 - protein, 38 aa, Artificial Sequence; identical to SEQ ID NO: 130
  compound Seq_179
  VARIANT 7: D-valine (v)
  VARIANT 12: K* denotes the modified lysine residue at X12, Ra denotes the albumin-binding moiety, Ra is "-gGlu-C(O)(CH2)16COOH
  VARIANT 23: 2-aminoisobutyric acid (Aib)
  MOD_RES 38: C-terminal amino acid residue is amidated as a primary amide

SEQ ID NO: 180 - protein, 38 aa, Artificial Sequence; identical to SEQ ID NO: 141
  compound Seq_180
  VARIANT 7: D-valine (v)
  VARIANT 12: K* denotes the modified lysine residue at X12, Ra denotes the albumin-binding moiety, Ra is "-gGlu-C(O)(CH2)16COOH
  VARIANT 23: 2-aminoisobutyric acid (Aib)
  MOD_RES 38: C-terminal amino acid residue is amidated as a primary amide

SEQ ID NO: 181 - protein, 38 aa, Artificial Sequence; identical to SEQ ID NO: 139
  compound Seq_181
  VARIANT 7: D-valine (v)
  VARIANT 12: K* denotes the modified lysine residue at X12, Ra denotes the albumin-binding moiety, Ra is "-gGlu-C(O)(CH2)16COOH
  MOD_RES 38: C-terminal amino acid residue is amidated as a primary amide

SEQ ID NO: 182 - protein, 38 aa, Artificial Sequence; identical to SEQ ID NO: 130
  compound Seq_182
  VARIANT 7: D-valine (v)
  VARIANT 12: K* denotes the modified lysine residue at X12, Ra denotes the albumin-binding moiety, Ra is "-C(O)(CH2)16COOH
  VARIANT 23: 2-aminoisobutyric acid (Aib)
  MOD_RES 38: C-terminal amino acid residue is amidated as a primary amide

SEQ ID NO: 183 - protein, 38 aa, Artificial Sequence; identical to SEQ ID NO: 141
  compound Seq_183
  VARIANT 7: D-valine (v)
  VARIANT 12: K* denotes the modified lysine residue at X12, Ra denotes the albumin-binding moiety, Ra is "-C(O)(CH2)16COOH
  VARIANT 23: 2-aminoisobutyric acid (Aib)
  MOD_RES 38: C-terminal amino acid residue is amidated as a primary amide

SEQ ID NO: 184 - protein, 38 aa, Artificial Sequence; identical to SEQ ID NO: 139
  compound Seq_184
  VARIANT 7: D-valine (v)
  VARIANT 12: K* denotes the modified lysine residue at X12, Ra denotes the albumin-binding moiety, Ra is "-C(O)(CH2)16COOH
  MOD_RES 38: C-terminal amino acid residue is amidated as a primary amide

SEQ ID NO: 185 - protein, 38 aa, Artificial Sequence
  compound Seq_185
  VARIANT 12: K* denotes the modified lysine residue at X12, Ra denotes the albumin-binding moiety, Ra is "-{AEEA}2-gGlu-C(O)(CH2)16COOH
  VARIANT 24: 2-aminoisobutyric acid (Aib)
  MOD_RES 38: C-terminal amino acid residue is amidated as a primary amide
IVLSLDVPIKLKQILLKQERQKKXRQKAETNKQILAQV

SEQ ID NO: 186 - protein, 38 aa, Artificial Sequence
  compound Seq_186
  VARIANT 1: isoleucine (I) or phenylalanine (F)
  VARIANT 2: valine (V) or threonine (T)
  VARIANT 7: valine (V) or D-valine (v)
  VARIANT 9: isoleucine (I) or threonine (T)
  VARIANT 10: lysine (K), glutamate (E), histidine (H) or glycine (G)
  VARIANT 11: isoleucine (I) or leucine (L)
  VARIANT 12: lysine (K), wherein the epsilon-amino group of the lysine side chain is covalently bound to an albumin-binding moiety
  VARIANT 13: glutamine (Q) or lysine (K)
  VARIANT 14: isoleucine (I), lysine (K) or 2-aminoisobutyric acid (Aib)
  VARIANT 16: leucine (L) or phenylalanine (F)
  VARIANT 17: glutamate (E) or lysine (K)
  VARIANT 19: alanine (A), glutamate (E) or glutamine (Q)
  VARIANT 20: lysine (K) or arginine (R)
  VARIANT 21: glutamine (Q) or lysine (K)
  VARIANT 22: lysine (K), arginine (R) or glutamate (E)
  VARIANT 23: lysine (K) or 2-aminoisobutyric acid (Aib)
  VARIANT 24: glutamine (Q), 2-aminoisobutyric acid (Aib), leucine (L) or glutamate (E)
  VARIANT 25: arginine (R), lysine (K) or 2-aminoisobutyric acid (Aib)
  VARIANT 26: alanine (A), glutamate (E), 2-aminoisobutyric acid (Aib) or glutamine (Q)
  VARIANT 27: glutamine (Q), 2-aminoisobutyric acid (Aib) or lysine (K)
  VARIANT 29: glutamate (E) or lysine (K)
  VARIANT 30: lysine (K) or threonine (T)
  VARIANT 31: asparagine (N) or alanine (A)
  VARIANT 32: lysine (K), alanine (A), valine (V), threonine (T), glutamate (E) or 2-aminoisobutyric acid (Aib)
  VARIANT 33: arginine (R), lysine (K) or glutamine (Q)
  VARIANT 34: isoleucine (I) or leucine (L)
  VARIANT 36: alanine (A) or glutamate (E)
  VARIANT 37: glutamine (Q) or arginine (R)
  VARIANT 38: isoleucine (I) or valine (V)
XXLSLDXPXXXXXXLXXQXXXXXXXXXAXXXXXXLXXX

SEQ ID NO: 187 - protein, 38 aa, Artificial Sequence
  >CRP-001 210819 Sequence Listing final_seq_187; AA; synthetic construct>
  VARIANT 7: D-valine (v)
  VARIANT 12: K* denotes the modified lysine residue at X12, Ra denotes the albumin-binding moiety, Ra is "--gGlu-C(O)(CH2)14COOH
  VARIANT 23: 2-aminoisobutyric acid (Aib)
  MOD_RES 38: C-terminal amino acid residue is amidated as a primary amide
IVLSLDVPIKLKQILLKQERQKXQREQAEKNKQILAQV

SEQ ID NO: 188 - protein, 38 aa, Artificial Sequence; identical to SEQ ID NO: 117
  >CRP-001 210819 Sequence Listing final_seq_188; AA; synthetic construct>
  VARIANT 7: D-valine (v)
  VARIANT 12: K* denotes the modified lysine residue at X12, Ra denotes the albumin-binding moiety, Ra is "--gGlu-C(O)(CH2)14COOH
  VARIANT 22: 2-aminoisobutyric acid (Aib)
  MOD_RES 38: C-terminal amino acid residue is amidated as a primary amide

SEQ ID NO: 189 - protein, 38 aa, Artificial Sequence; identical to SEQ ID NO: 119
  >CRP-001 210819 Sequence Listing final_seq_189; AA; synthetic construct>
  VARIANT 7: D-valine (v)
  VARIANT 12: K* denotes the modified lysine residue at X12, Ra denotes the albumin-binding moiety, Ra is "-gGlu-C(O)(CH2)14COOH
  VARIANT 24: 2-aminoisobutyric acid (Aib)
  MOD_RES 38: C-terminal amino acid residue is amidated as a primary amide

SEQ ID NO: 190 - protein, 38 aa, Artificial Sequence; identical to SEQ ID NO: 120
  >CRP-001 210819 Sequence Listing final_seq_190; AA; synthetic construct>
  VARIANT 7: D-valine (v)
  VARIANT 12: K* denotes the modified lysine residue at X12, Ra denotes the albumin-binding moiety, Ra is "-gGlu-C(O)(CH2)14COOH
  MOD_RES 38: C-terminal amino acid residue is amidated as a primary amide

SEQ ID NO: 191 - protein, 38 aa, Artificial Sequence; identical to SEQ ID NO: 121
  >CRP-001 210819 Sequence Listing final_seq_191; AA; synthetic construct>
  VARIANT 7: D-valine (v)
  VARIANT 12: K* denotes the modified lysine residue at X12, Ra denotes the albumin-binding moiety, Ra is "-gGlu-C(O)(CH2)14COOH
  MOD_RES 38: C-terminal amino acid residue is amidated as a primary amide

SEQ ID NO: 192 - protein, 38 aa, Artificial Sequence; identical to SEQ ID NO: 122
  >CRP-001 210819 Sequence Listing final_seq_192; AA; synthetic construct>
  VARIANT 7: D-valine (v)
  VARIANT 12: K* denotes the modified lysine residue at X12, Ra denotes the albumin-binding moiety, Ra is "-gGlu-C(O)(CH2)14COOH
  MOD_RES 38: C-terminal amino acid residue is amidated as a primary amide

SEQ ID NO: 193 - protein, 38 aa, Artificial Sequence; identical to SEQ ID NO: 148
  >CRP-001 210819 Sequence Listing final_seq_193; AA; synthetic construct>
  VARIANT 7: D-valine (v)
  VARIANT 12: K* denotes the modified lysine residue at X12, Ra denotes the albumin-binding moiety, Ra is "-gGlu-C(O)(CH2)14COOH
  VARIANT 24: 2-aminoisobutyric acid (Aib)
  MOD_RES 38: C-terminal amino acid residue is amidated as a primary amide

SEQ ID NO: 194 - protein, 38 aa, Artificial Sequence
  >CRP-001 210819 Sequence Listing final_seq_194; AA; synthetic construct>
  VARIANT 7: D-valine (v)
  VARIANT 12: K* denotes the modified lysine residue at X12, Ra denotes the albumin-binding moiety, Ra is "-gGlu-C(O)(CH2)14COOH
  VARIANT 24: 2-aminoisobutyric acid (Aib)
  MOD_RES 38: C-terminal amino acid residue is amidated as a primary amide
IVLSLDVPIGLKQILLKQERQKKXREQAETNKQILAQV

SEQ ID NO: 195 - protein, 38 aa, Artificial Sequence
  >CRP-001 210819 Sequence Listing final_seq_195; AA; synthetic construct>
  VARIANT 7: D-valine (v)
  VARIANT 12: K* denotes the modified lysine residue at X12, Ra denotes the albumin-binding moiety, Ra is "-gGlu-C(O)(CH2)14COOH
  VARIANT 24: 2-aminoisobutyric acid (Aib)
  MOD_RES 38: C-terminal amino acid residue is amidated as a primary amide
IVLSLDVPIGLKQILLKQERQKKXRQQAETNKRILERV

SEQ ID NO: 196 - protein, 38 aa, Artificial Sequence
  >CRP-001 210819 Sequence Listing final_seq_196; AA; synthetic construct>
  VARIANT 7: D-valine (v)
  VARIANT 12: K* denotes the modified lysine residue at X12, Ra denotes the albumin-binding moiety, Ra is "-gGlu-C(O)(CH2)14COOH
  VARIANT 24: 2-aminoisobutyric acid (Aib)
  MOD_RES 38: C-terminal amino acid residue is amidated as a primary amide
IVLSLDVPIGLKQILLKQERQKKXREQAEKNKRILERV

SEQ ID NO: 197 - protein, 38 aa, Artificial Sequence; identical to SEQ ID NO: 124
  >CRP-001 210819 Sequence Listing final_seq_197; AA; synthetic construct>
  VARIANT 7: D-valine (v)
  VARIANT 12: K* denotes the modified lysine residue at X12, Ra denotes the albumin-binding moiety, Ra is "-gGlu-C(O)(CH2)14COOH
  VARIANT 23: 2-aminoisobutyric acid (Aib)
  MOD_RES 38: C-terminal amino acid residue is amidated as a primary amide

SEQ ID NO: 198 - protein, 38 aa, Artificial Sequence; identical to SEQ ID NO: 187
  >CRP-001 210819 Sequence Listing final_seq_198; AA; synthetic construct>
  VARIANT 7: D-valine (v)
  VARIANT 12: K* denotes the modified lysine residue at X12, Ra denotes the albumin-binding moiety, Ra is "-{AEEA}2-gGlu-C(O)(CH2)14COOH
  VARIANT 23: 2-aminoisobutyric acid (Aib)
  MOD_RES 38: C-terminal amino acid residue is amidated as a primary amide

SEQ ID NO: 199 - protein, 38 aa, Artificial Sequence; identical to SEQ ID NO: 187
  >CRP-001 210819 Sequence Listing final_seq_199; AA; synthetic construct>
  VARIANT 7: D-valine (v)
  VARIANT 12: K* denotes the modified lysine residue at X12, Ra denotes the albumin-binding moiety, Ra is "-{AEEA}2-{gGLU}2-C(O)(CH2)14COOH
  VARIANT 23: 2-aminoisobutyric acid (Aib)
  MOD_RES 38: C-terminal amino acid residue is amidated as a primary amide

SEQ ID NO: 200 - protein, 38 aa, Artificial Sequence; identical to SEQ ID NO: 119
  >CRP-001 210819 Sequence Listing final_seq_200; AA; synthetic construct>
  VARIANT 7: D-valine (v)
  VARIANT 12: K* denotes the modified lysine residue at X12, Ra denotes the albumin-binding moiety, Ra is "-{AEEA}2-gGlu-C(O)(CH2)14COOH
  VARIANT 24: 2-aminoisobutyric acid (Aib)
  MOD_RES 38: C-terminal amino acid residue is amidated as a primary amide

SEQ ID NO: 201 - protein, 38 aa, Artificial Sequence; identical to SEQ ID NO: 119
  >CRP-001 210819 Sequence Listing final_seq_201; AA; synthetic construct>
  VARIANT 7: D-valine (v)
  VARIANT 12: K* denotes the modified lysine residue at X12, Ra denotes the albumin-binding moiety, Ra is "-{AEEA}2-{gGLU}2-C(O)(CH2)14COOH
  VARIANT 24: 2-aminoisobutyric acid (Aib)
  MOD_RES 38: C-terminal amino acid residue is amidated as a primary amide

SEQ ID NO: 202 - protein, 38 aa, Artificial Sequence; identical to SEQ ID NO: 194
  >CRP-001 210819 Sequence Listing final_seq_202; AA; synthetic construct>
  VARIANT 7: D-valine (v)
  VARIANT 12: K* denotes the modified lysine residue at X12, Ra denotes the albumin-binding moiety, Ra is "-{AEEA}2-gGlu-C(O)(CH2)14COOH
  VARIANT 24: 2-aminoisobutyric acid (Aib)
  MOD_RES 38: C-terminal amino acid residue is amidated as a primary amide

SEQ ID NO: 203 - protein, 38 aa, Artificial Sequence; identical to SEQ ID NO: 194
  >CRP-001 210819 Sequence Listing final_seq_203; AA; synthetic construct>
  VARIANT 7: D-valine (v)
  VARIANT 12: K* denotes the modified lysine residue at X12, Ra denotes the albumin-binding moiety, Ra is "-{AEEA}2-gGlu-C(O)(CH2)14COOH
  VARIANT 24: 2-aminoisobutyric acid (Aib)
  MOD_RES 38: C-terminal amino acid residue is amidated as a primary amide

SEQ ID NO: 204 - protein, 38 aa, Artificial Sequence; identical to SEQ ID NO: 187
  >CRP-001 210819 Sequence Listing final_seq_204; AA; synthetic construct>
  VARIANT 7: D-valine (v)
  VARIANT 12: K* denotes the modified lysine residue at X12, Ra denotes the albumin-binding moiety, Ra is "-gGlu-C(O)(CH2)14CH3
  VARIANT 23: 2-aminoisobutyric acid (Aib)
  MOD_RES 38: C-terminal amino acid residue is amidated as a primary amide

SEQ ID NO: 205 - protein, 38 aa, Artificial Sequence; identical to SEQ ID NO: 187
  >CRP-001 210819 Sequence Listing final_seq_205; AA; synthetic construct>
  VARIANT 7: D-valine (v)
  VARIANT 12: K* denotes the modified lysine residue at X12, Ra denotes the albumin-binding moiety, Ra is "-{AEEA}2-gGlu-C(O)(CH2)14CH3
  VARIANT 23: 2-aminoisobutyric acid (Aib)
  MOD_RES 38: C-terminal amino acid residue is amidated as a primary amide

SEQ ID NO: 206 - protein, 38 aa, Artificial Sequence; identical to SEQ ID NO: 187
  >CRP-001 210819 Sequence Listing final_seq_206; AA; synthetic construct>
  VARIANT 7: D-valine (v)
  VARIANT 12: K* denotes the modified lysine residue at X12, Ra denotes the albumin-binding moiety, Ra is "-{AEEA}2-{gGLU}2-C(O)(CH2)14CH3
  VARIANT 23: 2-aminoisobutyric acid (Aib)
  MOD_RES 38: C-terminal amino acid residue is amidated as a primary amide

SEQ ID NO: 207 - protein, 38 aa, Artificial Sequence; identical to SEQ ID NO: 148
  >CRP-001 210819 Sequence Listing final_seq_207; AA; synthetic construct>
  VARIANT 7: D-valine (v)
  VARIANT 12: K* denotes the modified lysine residue at X12, Ra denotes the albumin-binding moiety, Ra is "-gGlu-C(O)(CH2)14CH3
  VARIANT 24: 2-aminoisobutyric acid (Aib)
  MOD_RES 38: C-terminal amino acid residue is amidated as a primary amide

SEQ ID NO: 208 - protein, 38 aa, Artificial Sequence; identical to SEQ ID NO: 117
  >CRP-001 210819 Sequence Listing final_seq_208; AA; synthetic construct>
  VARIANT 7: D-valine (v)
  VARIANT 12: K* denotes the modified lysine residue at X12, Ra denotes the albumin-binding moiety, Ra is "-gGlu-C(O)(CH2)14CH3
  VARIANT 23: 2-aminoisobutyric acid (Aib)
  MOD_RES 38: C-terminal amino acid residue is amidated as a primary amide

SEQ ID NO: 209 - protein, 38 aa, Artificial Sequence; identical to SEQ ID NO: 119
  >CRP-001 210819 Sequence Listing final_seq_209; AA; synthetic construct>
  VARIANT 7: D-valine (v)
  VARIANT 12: K* denotes the modified lysine residue at X12, Ra denotes the albumin-binding moiety, Ra is "-gGlu-C(O)(CH2)14CH3
  VARIANT 24: 2-aminoisobutyric acid (Aib)
  MOD_RES 38: C-terminal amino acid residue is amidated as a primary amide

SEQ ID NO: 210 - protein, 38 aa, Artificial Sequence; identical to SEQ ID NO: 119
  >CRP-001 210819 Sequence Listing final_seq_210; AA; synthetic construct>
  VARIANT 7: D-valine (v)
  VARIANT 12: K* denotes the modified lysine residue at X12, Ra denotes the albumin-binding moiety, Ra is "-{AEEA}2-gGlu-C(O)(CH2)14CH3
  VARIANT 24: 2-aminoisobutyric acid (Aib)
  MOD_RES 38: C-terminal amino acid residue is amidated as a primary amide

SEQ ID NO: 211 - protein, 38 aa, Artificial Sequence; identical to SEQ ID NO: 119
  >CRP-001 210819 Sequence Listing final_seq_211; AA; synthetic construct>
  VARIANT 7: D-valine (v)
  VARIANT 12: K* denotes the modified lysine residue at X12, Ra denotes the albumin-binding moiety, Ra is "-{AEEA}2-{gGLU}2-C(O)(CH2)14CH3
  VARIANT 24: 2-aminoisobutyric acid (Aib)
  MOD_RES 38: C-terminal amino acid residue is amidated as a primary amide

SEQ ID NO: 212 - protein, 38 aa, Artificial Sequence; identical to SEQ ID NO: 120
  >CRP-001 210819 Sequence Listing final_seq_212; AA; synthetic construct>
  VARIANT 7: D-valine (v)
  VARIANT 12: K* denotes the modified lysine residue at X12, Ra denotes the albumin-binding moiety, Ra is "-gGlu-C(O)(CH2)14CH3
  MOD_RES 38: C-terminal amino acid residue is amidated as a primary amide

SEQ ID NO: 213 - protein, 38 aa, Artificial Sequence; identical to SEQ ID NO: 121
  >CRP-001 210819 Sequence Listing final_seq_213; AA; synthetic construct>
  VARIANT 7: D-valine (v)
  VARIANT 12: K* denotes the modified lysine residue at X12, Ra denotes the albumin-binding moiety, Ra is "-gGlu-C(O)(CH2)14CH3
  MOD_RES 38: C-terminal amino acid residue is amidated as a primary amide

SEQ ID NO: 214 - protein, 38 aa, Artificial Sequence; identical to SEQ ID NO: 122
  >CRP-001 210819 Sequence Listing final_seq_214; AA; synthetic construct>
  VARIANT 7: D-valine (v)
  VARIANT 12: K* denotes the modified lysine residue at X12, Ra denotes the albumin-binding moiety, Ra is "-gGlu-C(O)(CH2)14CH3
  MOD_RES 38: C-terminal amino acid residue is amidated as a primary amide

SEQ ID NO: 215 - protein, 38 aa, Artificial Sequence; identical to SEQ ID NO: 194
  >CRP-001 210819 Sequence Listing final_seq_215; AA; synthetic construct>
  VARIANT 7: D-valine (v)
  VARIANT 12: K* denotes the modified lysine residue at X12, Ra denotes the albumin-binding moiety, Ra is "-gGlu-C(O)(CH2)14CH3
  VARIANT 24: 2-aminoisobutyric acid (Aib)
  MOD_RES 38: C-terminal amino acid residue is amidated as a primary amide

SEQ ID NO: 216 - protein, 38 aa, Artificial Sequence; identical to SEQ ID NO: 194
  >CRP-001 210819 Sequence Listing final_seq_216; AA; synthetic construct>
  VARIANT 7: D-valine (v)
  VARIANT 12: K* denotes the modified lysine residue at X12, Ra denotes the albumin-binding moiety, Ra is "-gGlu-C(O)(CH2)14CH3
  VARIANT 24: 2-aminoisobutyric acid (Aib)
  MOD_RES 38: C-terminal amino acid residue is amidated as a primary amide

SEQ ID NO: 217 - protein, 38 aa, Artificial Sequence; identical to SEQ ID NO: 194
  >CRP-001 210819 Sequence Listing final_seq_217; AA; synthetic construct>
  VARIANT 7: D-valine (v)
  VARIANT 12: K* denotes the modified lysine residue at X12, Ra denotes the albumin-binding moiety, Ra is "-gGlu-C(O)(CH2)14CH3
  VARIANT 24: 2-aminoisobutyric acid (Aib)
  MOD_RES 38: C-terminal amino acid residue is amidated as a primary amide

SEQ ID NO: 218 - protein, 38 aa, Artificial Sequence; identical to SEQ ID NO: 196
  >CRP-001 210819 Sequence Listing final_seq_218; AA; synthetic construct>
  VARIANT 7: D-valine (v)
  VARIANT 12: K* denotes the modified lysine residue at X12, Ra denotes the albumin-binding moiety, Ra is "-gGlu-C(O)(CH2)14CH3
  VARIANT 24: 2-aminoisobutyric acid (Aib)
  MOD_RES 38: C-terminal amino acid residue is amidated as a primary amide

SEQ ID NO: 219 - protein, 38 aa, Artificial Sequence; identical to SEQ ID NO: 124
  >CRP-001 210819 Sequence Listing final_seq_219; AA; synthetic construct>
  VARIANT 7: D-valine (v)
  VARIANT 12: K* denotes the modified lysine residue at X12, Ra denotes the albumin-binding moiety, Ra is "-gGlu-C(O)(CH2)14CH3
  VARIANT 23: 2-aminoisobutyric acid (Aib)
  MOD_RES 38: C-terminal amino acid residue is amidated as a primary amide

SEQ ID NO: 220 - protein, 38 aa, Artificial Sequence; identical to SEQ ID NO: 195
  >CRP-001 210819 Sequence Listing final_seq_220; AA; synthetic construct>
  VARIANT 7: D-valine (v)
  VARIANT 12: K* denotes the modified lysine residue at X12, Ra denotes the albumin-binding moiety, Ra is "-gGlu-C(O)(CH2)14CH3
  VARIANT 24: 2-aminoisobutyric acid (Aib)
  MOD_RES 38: C-terminal amino acid residue is amidated as a primary amide

SEQ ID NO: 221 - protein, 38 aa, Artificial Sequence
  >CRP-001 210819 Sequence Listing final_seq_221; AA; synthetic construct>
  VARIANT 7: D-valine (v)
  VARIANT 12: K* denotes the modified lysine residue at X12, Ra denotes the albumin-binding moiety, Ra is "-gGlu-C(O)(CH2)14COOH
  MOD_RES 38: C-terminal amino acid residue is amidated as a primary amide
IVLSLDVPTKLKQKLLKQERQRKEREQAEKNARILARV

SEQ ID NO: 222 - protein, 38 aa, Artificial Sequence
  >CRP-001 210819 Sequence Listing final_seq_222; AA; synthetic construct>
  VARIANT 7: D-valine (v)
  VARIANT 12: K* denotes the modified lysine residue at X12, Ra denotes the albumin-binding moiety, Ra is "-gGlu-C(O)(CH2)14COOH
  MOD_RES 38: C-terminal amino acid residue is amidated as a primary amide
IVLSLDVPTKLKQKLLKQERQRKEREQAEKNVRILERV

SEQ ID NO: 223 - protein, 38 aa, Artificial Sequence
  >CRP-001 210819 Sequence Listing final_seq_223; AA; synthetic construct>
  VARIANT 7: D-valine (v)
  VARIANT 12: K* denotes the modified lysine residue at X12, Ra denotes the albumin-binding moiety, Ra is "-gGlu-C(O)(CH2)14CH3
  MOD_RES 38: C-terminal amino acid residue is amidated as a primary amide
IVLSLDVPTKLKQKLLKQERQRKEREQAEKNKRILERV

SEQ ID NO: 224 - protein, 38 aa, Artificial Sequence; identical to SEQ ID NO: 47
  >CRP-001 210819 Sequence Listing final_seq_224; AA; synthetic construct>
  VARIANT 7: D-valine (v)
  VARIANT 12: K* denotes the modified lysine residue at X12, Ra denotes the albumin-binding moiety, Ra is "-{AEEA}2-gGlu-C(O)(CH2)18COOH
  VARIANT 23: 2-aminoisobutyric acid (Aib)
  MOD_RES 38: C-terminal amino acid residue is amidated as a primary amide

SEQ ID NO: 225 - protein, 38 aa, Artificial Sequence
  >CRP-001 210819 Sequence Listing final_seq_225; AA; synthetic construct>
  VARIANT 7: D-valine (v)
  VARIANT 12: K* denotes the modified lysine residue at X12, Ra denotes the albumin-binding moiety, Ra is "-gGlu-C(O)(CH2)14CH3
  VARIANT 27: 2-aminoisobutyric acid (Aib)
  MOD_RES 38: C-terminal amino acid residue is amidated as a primary amide
IVLSLDVPTKLKQKLLKQERQRKEREXAEKNKRILERV

SEQ ID NO: 226 - protein, 38 aa, Artificial Sequence
  >CRP-001 210819 Sequence Listing final_seq_226; AA; synthetic construct>
  VARIANT 7: D-valine (v)
  VARIANT 12: K* denotes the modified lysine residue at X12, Ra denotes the albumin-binding moiety, Ra is "-gGlu-C(O)(CH2)14CH3
  MOD_RES 38: C-terminal amino acid residue is amidated as a primary amide
IVLSLDVPIGLKQKLLKQQRQRKERQQAEKNKRILERV

SEQ ID NO: 227 - protein, 38 aa, Artificial Sequence
  >CRP-001 210819 Sequence Listing final_seq_227; AA; synthetic construct>
  VARIANT 7: D-valine (v)
  VARIANT 12: K* denotes the modified lysine residue at X12, Ra denotes the albumin-binding moiety, Ra is "-gGlu-C(O)(CH2)14CH3
  MOD_RES 38: C-terminal amino acid residue is amidated as a primary amide
IVLSLDVPIKLKQKLLKQQRQRKERQQAEKNKRILERV